European Patent Application EP 4 592 306 A2, published July 30, 2025. Title: RNA CONSTRUCTS AND USES THEREOF. Applicant: BIONTECH SE. Application EP, filed April 22, 2021. The sequence listing filed with the application follows.

SEQUENCE LISTING (46 sequences)

SEQ ID NO: 1-7 - skipped (7 entries)

SEQ ID NO: 8 - RNA, 20 nt, synthetic construct
  misc_feature 1..20: note = Description of Artificial Sequence: Synthetic oligonucleotide
  source 1..20: mol_type = other RNA
gagtcgctagccgcgtcgct

SEQ ID NO: 9 - protein, 1273 aa, synthetic construct
  REGION 1..1273: note = Description of Artificial Sequence: Synthetic polypeptide
MFVFLVLLPLVSSQCVNLTTRTQLPPAYTNSFTRGVYYPDKVFRSSVLHSTQDLFLPFFSNVTWFHAIHVSGTNGTKRFDNPVLPFNDGVYFASTEKSNIIRGWIFGTTLDSKTQSLLIVNNATNVVIKVCEFQFCNDPFLGVYYHKNNKSWMESEFRVYSSANNCTFEYVSQPFLMDLEGKQGNFKNLREFVFKNIDGYFKIYSKHTPINLVRDLPQGFSALEPLVDLPIGINITRFQTLLALHRSYLTPGDSSSGWTAGAAAYYVGYLQPRTFLLKYNENGTITDAVDCALDPLSETKCTLKSFTVEKGIYQTSNFRVQPTESIVRFPNITNLCPFGEVFNATRFASVYAWNRKRISNCVADYSVLYNSASFSTFKCYGVSPTKLNDLCFTNVYADSFVIRGDEVRQIAPGQTGKIADYNYKLPDDFTGCVIAWNSNNLDSKVGGNYNYLYRLFRKSNLKPFERDISTEIYQAGSTPCNGVEGFNCYFPLQSYGFQPTNGVGYQPYRVVVLSFELLHAPATVCGPKKSTNLVKNKCVNFNFNGLTGTGVLTESNKKFLPFQQFGRDIADTTDAVRDPQTLEILDITPCSFGGVSVITPGTNTSNQVAVLYQDVNCTEVPVAIHADQLTPTWRVYSTGSNVFQTRAGCLIGAEHVNNSYECDIPIGAGICASYQTQTNSPRRARSVASQSIIAYTMSLGAENSVAYSNNSIAIPTNFTISVTTEILPVSMTKTSVDCTMYICGDSTECSNLLLQYGSFCTQLNRALTGIAVEQDKNTQEVFAQVKQIYKTPPIKDFGGFNFSQILPDPSKPSKRSFIEDLLFNKVTLADAGFIKQYGDCLGDIAARDLICAQKFNGLTVLPPLLTDEMIAQYTSALLAGTITSGWTFGAGAALQIPFAMQMAYRFNGIGVTQNVLYENQKLIANQFNSAIGKIQDSLSSTASALGKLQDVVNQNAQALNTLVKQLSSNFGAISSVLNDILSRLDPPEAEVQIDRLITGRLQSLQTYVTQQLIRAAEIRASANLAATKMSECVLGQSKRVDFCGKGYHLMSFPQSAPHGVVFLHVTYVPAQEKNFTTAPAICHDGKAHFPREGVFVSNGTHWFVTQRNFYEPQIITTDNTFVSGNCDVVIGIVNNTVYDPLQPELDSFKEELDKYFKNHTSPDVDLGDISGINASVVNIQKEIDRLNEVAKNLNESLIDLQELGKYEQYIKWPWYIWLGFIAGLIAIVMVTIMLCCMTSCCSCLKGCCSCGSCCKFDEDDSEPVLKGVKLHYT

SEQ ID NO: 10 - RNA, 4283 nt, synthetic construct
  misc_feature 1..4283: note = Description of Artificial Sequence: Synthetic polynucleotide
  source 1..4283: mol_type = other RNA
agaataaactagtattcttctggtccccacagactcagagagaacccgccaccatgttcgtgttcctggtgctgctgcctctggtgtccagccagtgtgtgaacctgaccaccagaacacagctgcctccagcctacaccaacagctttaccagaggcgtgtactaccccgacaaggtgttcagatccagcgtgctgcactctacccaggacctgttcctgcctttcttcagcaacgtgacctggttccacgccatccacgtgtccggcaccaatggcaccaagagattcgacaaccccgtgctgcccttcaacgacggggtgtactttgccagcaccgagaagtccaacatcatcagaggctggatcttcggcaccacactggacagcaagacccagagcctgctgatcgtgaacaacgccaccaacgtggtcatcaaagtgtgcgagttccagttctgcaacgaccccttcctgggcgtctactaccacaagaacaacaagagctggatggaaagcgagttccgggtgtacagcagcgccaacaactgcaccttcgagtacgtgtcccagcctttcctgatggacctggaaggcaagcagggcaacttcaagaacctgcgcgagttcgtgtttaagaacatcgacggctacttcaagatctacagcaagcacacccctatcaacctcgtgcgggatctgcctcagggcttctctgctctggaacccctggtggatctgcccatcggcatcaacatcacccggtttcagacactgctggccctgcacagaagctacctgacacctggcgatagcagcagcggatggacagctggtgccgccgcttactatgtgggctacctgcagcctagaaccttcctgctgaagtacaacgagaacggcaccatcaccgacgccgtggattgtgctctggatcctctgagcgagacaaagtgcaccctgaagtccttcaccgtggaaaagggcatctaccagaccagcaacttccgggtgcagcccaccgaatccatcgtgcggttccccaatatcaccaatctgtgccccttcggcgaggtgttcaatgccaccagattcgcctctgtgtacgcctggaaccggaagcggatcagcaattgcgtggccgactactccgtgctgtacaactccgccagcttcagcaccttcaagtgctacggcgtgtcccctaccaagctgaacgacctgtgcttcacaaacgtgtacgccgacagcttcgtgatccggggagatgaagtgcggcagattgcccctggacagacaggcaagatcgccgactacaactacaagctgcccgacgacttcaccggctgtgtgattgcctggaacagcaacaacctggactccaaagtcggcggcaactacaattacctgtaccggctgttccggaagtccaatctgaagcccttcgagcgggacatctccaccgagatctatcaggccggcagcaccccttgtaacggcgtggaaggcttcaactgctacttcccactgcagtcctacggctttcagcccacaaatggcgtgggctatcagccctacagagtggtggtgctgagcttcgaactgctgcatgcccctgccacagtgtgcggccctaagaaaagcaccaatctcgtgaagaacaaatgcgtgaacttcaacttcaacggcctgaccggcaccggcgtgctgacagagagcaacaagaagttcctgccattccagcagtttggccgggatatcgccgataccacagacgccgttagagatccccagacactggaaatcctggacatcaccccttgcagcttcggcggagtgtctgtgatcacccctggcaccaacaccagcaatcaggtggcagtgctgtaccaggacgtgaactgtaccgaagtgcccgtggccattcacgccgatcagctgacacctacatggcgggtgtactccaccggcagcaatgtgtttcagaccagagccggctgtctgatcggagccgagcacgtgaacaatagctacgagtgcgacatccccatcggcgctggaatctgcgccagctaccagacacagacaaacagccctcggagagccagaagcgtggccagccagagcatcattgcctacacaatgtctctgggcgccgagaacagcgtggcctactccaacaactctatcgctatccccaccaacttcaccatcagcgtgaccacagagatcctgcctgtgtccatgaccaagaccagcgtggactgcaccatgtacatctgcggcgattccaccgagtgctccaacctgctgctgcagtacggcagcttctgcacccagctgaatagagccctgacagggatcgccgtggaacaggacaagaacacccaagaggtgttcgcccaagtgaagcagatctacaagacccctcctatcaaggacttcggcggcttcaatttcagccagattctgcccgatcctagcaagcccagcaagcggagcttcatcgaggacctgctgttcaacaaagtgacactggccgacgccggcttcatcaagcagtatggcgattgtctgggcgacattgccgccagggatctgatttgcgcccagaagtttaacggactgacagtgctgcctcctctgctgaccgatgagatgatcgcccagtacacatctgccctgctggccggcacaatcacaagcggctggacatttggagcaggcgccgctctgcagatcccctttgctatgcagatggcctaccggttcaacggcatcggagtgacccagaatgtgctgtacgagaaccagaagctgatcgccaaccagttcaacagcgccatcggcaagatccaggacagcctgagcagcacagcaagcgccctgggaaagctgcaggacgtggtcaaccagaatgcccaggcactgaacaccctggtcaagcagctgtcctccaacttcggcgccatcagctctgtgctgaacgatatcctgagcagactggaccctcctgaggccgaggtgcagatcgacagactgatcacaggcagactgcagagcctccagacatacgtgacccagcagctgatcagagccgccgagattagagcctctgccaatctggccgccaccaagatgtctgagtgtgtgctgggccagagcaagagagtggacttttgcggcaagggctaccacctgatgagcttccctcagtctgcccctcacggcgtggtgtttctgcacgtgacatatgtgcccgctcaagagaagaatttcaccaccgctccagccatctgccacgacggcaaagcccactttcctagagaaggcgtgttcgtgtccaacggcacccattggttcgtgacacagcggaacttctacgagccccagatcatcaccaccgacaacaccttcgtgtctggcaactgcgacgtcgtgatcggcattgtgaacaataccgtgtacgaccctctgcagcccgagctggacagcttcaaagaggaactggacaagtactttaagaaccacacaagccccgacgtggacctgggcgatatcagcggaatcaatgccagcgtcgtgaacatccagaaagagatcgaccggctgaacgaggtggccaagaatctgaacgagagcctgatcgacctgcaagaactggggaagtacgagcagtacatcaagtggccctggtacatctggctgggctttatcgccggactgattgccatcgtgatggtcacaatcatgctgtgttgcatgaccagctgctgtagctgcctgaagggctgttgtagctgtggcagctgctgcaagttcgacgaggacgattctgagcccgtgctgaagggcgtgaaactgcactacacatgatgactcgagctggtactgcatgcacgcaatgctagctgcccctttcccgtcctgggtaccccgagtctcccccgacctcgggtcccaggtatgctcccacctccacctgccccactcaccacctctgctagttccagacacctcccaagcacgcagcaatgcagctcaaaacgcttagcctagccacacccccacgggaaacagcagtgattaacctttagcaataaacgaaagtttaactaagctatactaaccccagggttggtcaatttcgtgccagccacaccctggagctagcaaaaaaaaaaaaaaaaaaaaaaaaaaaaaagcatatgactaaaaaaaaaaaaaaaaaaaaaaaaaaaaaaaaaaaaaaaaaaaaaaaaaaaaaaaaaaaaaaaaaaaaaa

SEQ ID NO: 11 - RNA, 47 nt, synthetic construct
  misc_feature 1..47: note = Description of Artificial Sequence: Synthetic oligonucleotide
  source 1..47: mol_type = other RNA
agaataaactagtattcttctggtccccacagactcagagagaaccc

SEQ ID NO: 12 - RNA, 42 nt, Homo sapiens
  source 1..42: mol_type = other RNA
aaactagtattcttctggtccccacagactcagagagaaccc

SEQ ID NO: 13 - RNA, 278 nt, synthetic construct
  misc_feature 1..278: note = Description of Artificial Sequence: Synthetic polynucleotide
  source 1..278: mol_type = other RNA
ctggtactgcatgcacgcaatgctagctgcccctttcccgtcctgggtaccccgagtctcccccgacctcgggtcccaggtatgctcccacctccacctgccccactcaccacctctgctagttccagacacctcccaagcacgcagcaatgcagctcaaaacgcttagcctagccacacccccacgggaaacagcagtgattaacctttagcaataaacgaaagtttaactaagctatactaaccccagggttggtcaatttcgtgccagccacacc

SEQ ID NO: 14 - RNA, 110 nt, synthetic construct
  misc_feature 1..110: note = Description of Artificial Sequence: Synthetic polynucleotide
  source 1..110: mol_type = other RNA
aaaaaaaaaaaaaaaaaaaaaaaaaaaaaagcatatgactaaaaaaaaaaaaaaaaaaaaaaaaaaaaaaaaaaaaaaaaaaaaaaaaaaaaaaaaaaaaaaaaaaaaaa

SEQ ID NO: 15 - RNA, 458 nt, synthetic construct
  misc_feature 1..458: note = Description of Artificial Sequence: Synthetic polynucleotide
  source 1..458: mol_type = other RNA
agaataaactagtattcttctggtccccacagactcagagagaacccgccaccctcgagctggtactgcatgcacgcaatgctagctgcccctttcccgtcctgggtaccccgagtctcccccgacctcgggtcccaggtatgctcccacctccacctgccccactcaccacctctgctagttccagacacctcccaagcacgcagcaatgcagctcaaaacgcttagcctagccacacccccacgggaaacagcagtgattaacctttagcaataaacgaaagtttaactaagctatactaaccccagggttggtcaatttcgtgccagccacaccctggagctagcaaaaaaaaaaaaaaaaaaaaaaaaaaaaaagcatatgactaaaaaaaaaaaaaaaaaaaaaaaaaaaaaaaaaaaaaaaaaaaaaaaaaaaaaaaaaaaaaaaaaaaaaa

SEQ ID NO: 16 - RNA, 4283 nt, synthetic construct; identical to SEQ ID NO: 10
  misc_feature 1..4283: note = Description of Artificial Sequence: Synthetic polynucleotide
  source 1..4283: mol_type = other RNA

SEQ ID NO: 17 - protein, 1273 aa, Severe acute respiratory syndrome-related coronavirus
MFVFLVLLPLVSSQCVNLTTRTQLPPAYTNSFTRGVYYPDKVFRSSVLHSTQDLFLPFFSNVTWFHAIHVSGTNGTKRFDNPVLPFNDGVYFASTEKSNIIRGWIFGTTLDSKTQSLLIVNNATNVVIKVCEFQFCNDPFLGVYYHKNNKSWMESEFRVYSSANNCTFEYVSQPFLMDLEGKQGNFKNLREFVFKNIDGYFKIYSKHTPINLVRDLPQGFSALEPLVDLPIGINITRFQTLLALHRSYLTPGDSSSGWTAGAAAYYVGYLQPRTFLLKYNENGTITDAVDCALDPLSETKCTLKSFTVEKGIYQTSNFRVQPTESIVRFPNITNLCPFGEVFNATRFASVYAWNRKRISNCVADYSVLYNSASFSTFKCYGVSPTKLNDLCFTNVYADSFVIRGDEVRQIAPGQTGKIADYNYKLPDDFTGCVIAWNSNNLDSKVGGNYNYLYRLFRKSNLKPFERDISTEIYQAGSTPCNGVEGFNCYFPLQSYGFQPTNGVGYQPYRVVVLSFELLHAPATVCGPKKSTNLVKNKCVNFNFNGLTGTGVLTESNKKFLPFQQFGRDIADTTDAVRDPQTLEILDITPCSFGGVSVITPGTNTSNQVAVLYQDVNCTEVPVAIHADQLTPTWRVYSTGSNVFQTRAGCLIGAEHVNNSYECDIPIGAGICASYQTQTNSPRRARSVASQSIIAYTMSLGAENSVAYSNNSIAIPTNFTISVTTEILPVSMTKTSVDCTMYICGDSTECSNLLLQYGSFCTQLNRALTGIAVEQDKNTQEVFAQVKQIYKTPPIKDFGGFNFSQILPDPSKPSKRSFIEDLLFNKVTLADAGFIKQYGDCLGDIAARDLICAQKFNGLTVLPPLLTDEMIAQYTSALLAGTITSGWTFGAGAALQIPFAMQMAYRFNGIGVTQNVLYENQKLIANQFNSAIGKIQDSLSSTASALGKLQDVVNQNAQALNTLVKQLSSNFGAISSVLNDILSRLDKVEAEVQIDRLITGRLQSLQTYVTQQLIRAAEIRASANLAATKMSECVLGQSKRVDFCGKGYHLMSFPQSAPHGVVFLHVTYVPAQEKNFTTAPAICHDGKAHFPREGVFVSNGTHWFVTQRNFYEPQIITTDNTFVSGNCDVVIGIVNNTVYDPLQPELDSFKEELDKYFKNHTSPDVDLGDISGINASVVNIQKEIDRLNEVAKNLNESLIDLQELGKYEQYIKWPWYIWLGFIAGLIAIVMVTIMLCCMTSCCSCLKGCCSCGSCCKFDEDDSEPVLKGVKLHYT

SEQ ID NO: 18 - RNA, 3819 nt, Severe acute respiratory syndrome-related coronavirus
  source 1..3819: mol_type = other RNA
atgtttgtgtttcttgtgctgctgcctcttgtgtcttctcagtgtgtgaatttgacaacaagaacacagctgccaccagcttatacaaattcttttaccagaggagtgtattatcctgataaagtgtttagatcttctgtgctgcacagcacacaggacctgtttctgccattttttagcaatgtgacatggtttcatgcaattcatgtgtctggaacaaatggaacaaaaagatttgataatcctgtgctgccttttaatgatggagtgtattttgcttcaacagaaaagtcaaatattattagaggatggatttttggaacaacactggattctaaaacacagtctctgctgattgtgaataatgcaacaaatgtggtgattaaagtgtgtgaatttcagttttgtaatgatccttttctgggagtgtattatcacaaaaataataaatcttggatggaatctgaatttagagtgtattcctctgcaaataattgtacatttgaatatgtgtctcagccttttctgatggatctggaaggaaaacagggcaattttaaaaatctgagagaatttgtgtttaaaaatattgatggatattttaaaatttattctaaacacacaccaattaatttagtgagagatctgcctcagggattttctgctctggaacctctggtggatctgccaattggcattaatattacaagatttcagacactgctggctctgcacagatcttatctgacacctggagattcttcttctggatggacagccggagctgcagcttattatgtgggctatctgcagccaagaacatttctgctgaaatataatgaaaatggaacaattacagatgctgtggattgtgctctggatcctctgtctgaaacaaaatgtacattaaaatcttttacagtggaaaaaggcatttatcagacatctaattttagagtgcagccaacagaatctattgtgagatttccaaatattacaaatctgtgtccatttggagaagtgtttaatgcaacaagatttgcatctgtgtatgcatggaatagaaaaagaatttctaattgtgtggctgattattctgtgctgtataatagtgcttctttttccacatttaaatgttatggagtgtctccaacaaaattaaatgatttatgttttacaaatgtgtatgctgattcttttgtgatcagaggtgatgaagtgagacagattgcccccggacagacaggaaaaattgctgattacaattacaaactgcctgatgattttacaggatgtgtgattgcttggaattctaataatttagattctaaagtgggaggaaattacaattatctgtacagactgtttagaaaatcaaatctgaaaccttttgaaagagatatttcaacagaaatttatcaggctggatcaacaccttgtaatggagtggaaggatttaattgttattttccattacagagctatggatttcagccaaccaatggtgtgggatatcagccatatagagtggtggtgctgtcttttgaactgctgcatgcacctgcaacagtgtgtggacctaaaaaatctacaaatttagtgaaaaataaatgtgtgaattttaattttaatggattaacaggaacaggagtgctgacagaatctaataaaaaatttctgccttttcagcagtttggcagagatattgcagataccacagatgcagtgagagatcctcagacattagaaattctggatattacaccttgttcttttgggggtgtgtctgtgattacacctggaacaaatacatctaatcaggtggctgtgctgtatcaggatgtgaattgtacagaagtgccagtggcaattcatgcagatcagctgacaccaacatggagagtgtattctacaggatctaatgtgtttcagacaagagcaggatgtctgattggagcagaacatgtgaataattcttatgaatgtgatattccaattggagcaggcatttgtgcatcttatcagacacagacaaattccccaaggagagcaagatctgtggcatctcagtctattattgcatacaccatgtctctgggagcagaaaattctgtggcatattctaataattctattgctattccaacaaattttaccatttctgtgacaacagaaattttacctgtgtctatgacaaaaacatctgtggattgtaccatgtacatttgtggagattctacagaatgttctaatctgctgctgcagtatggatctttttgtacacagctgaatagagctttaacaggaattgctgtggaacaggataaaaatacacaggaagtgtttgctcaggtgaaacagatttacaaaacaccaccaattaaagattttggaggatttaattttagccagattctgcctgatccttctaaaccttctaaaagatcttttattgaagatctgctgtttaataaagtgacactggcagatgcaggatttattaaacagtatggagattgcctgggtgatattgctgcaagagatctgatttgtgctcagaaatttaatggactgacagtgctgcctcctctgctgacagatgaaatgattgctcagtacacatctgctttactggctggaacaattacaagcggatggacatttggagctggagctgctctgcagattccttttgcaatgcagatggcttacagatttaatggaattggagtgacacagaatgtgttatatgaaaatcagaaactgattgcaaatcagtttaattctgcaattggcaaaattcaggattctctgtcttctacagcttctgctctgggaaaactgcaggatgtggtgaatcagaatgcacaggcactgaatactctggtgaaacagctgtctagcaattttggggcaatttcttctgtgctgaatgatattctgtctagactggataaagtggaagctgaagtgcagattgatagactgatcacaggaagactgcagtctctgcagacttatgtgacacagcagctgattagagctgctgaaattagagcttctgctaatctggctgctacaaaaatgtctgaatgtgtgctgggacagtcaaaaagagtggatttttgtggaaaaggatatcatctgatgtcttttccacagtctgctccacatggagtggtgtttttacatgtgacatatgtgccagcacaggaaaagaattttaccacagcaccagcaatttgtcatgatggaaaagcacattttccaagagaaggagtgtttgtgtctaatggaacacattggtttgtgacacagagaaatttttatgaacctcagattattacaacagataatacatttgtgtcaggaaattgtgatgtggtgattggaattgtgaataatacagtgtatgatccactgcagccagaactggattcttttaaagaagaactggataaatattttaaaaatcacacatctcctgatgtggatttaggagatatttctggaatcaatgcatctgtggtgaatattcagaaagaaattgatagactgaatgaagtggccaaaaatctgaatgaatctctgattgatctgcaggaacttggaaaatatgaacagtacattaaatggccttggtacatttggcttggatttattgcaggattaattgcaattgtgatggtgacaattatgttatgttgtatgacatcatgttgttcttgtttaaaaggatgttgttcttgtggaagctgttgtaaatttgatgaagatgattctgaacctgtgttaaaaggagtgaaattgcattacaca

SEQ ID NO: 19 - protein, 218 aa, synthetic construct
  REGION 1..218: note = Description of Artificial Sequence: Synthetic polypeptide
MFVFLVLLPLVSSQCVVRFPNITNLCPFGEVFNATRFASVYAWNRKRISNCVADYSVLYNSASFSTFKCYGVSPTKLNDLCFTNVYADSFVIRGDEVRQIAPGQTGKIADYNYKLPDDFTGCVIAWNSNNLDSKVGGNYNYLYRLFRKSNLKPFERDISTEIYQAGSTPCNGVEGFNCYFPLQSYGFQPTNGVGYQPYRVVVLSFELLHAPATVCGPK

SEQ ID NO: 20 - RNA, 654 nt, synthetic construct
  misc_feature 1..654: note = Description of Artificial Sequence: Synthetic polynucleotide
  source 1..654: mol_type = other RNA
atgtttgtgtttcttgtgctgctgcctcttgtgtcttctcagtgtgtggtgagatttccaaatattacaaatctgtgtccatttggagaagtgtttaatgcaacaagatttgcatctgtgtatgcatggaatagaaaaagaatttctaattgtgtggctgattattctgtgctgtataatagtgcttctttttccacatttaaatgttatggagtgtctccaacaaaattaaatgatttatgttttacaaatgtgtatgctgattcttttgtgatcagaggtgatgaagtgagacagattgcccccggacagacaggaaaaattgctgattacaattacaaactgcctgatgattttacaggatgtgtgattgcttggaattctaataatttagattctaaagtgggaggaaattacaattatctgtacagactgtttagaaaatcaaatctgaaaccttttgaaagagatatttcaacagaaatttatcaggctggatcaacaccttgtaatggagtggaaggatttaattgttattttccattacagagctatggatttcagccaaccaatggtgtgggatatcagccatatagagtggtggtgctgtcttttgaactgctgcatgcacctgcaacagtgtgtggacctaaa

SEQ ID NO: 21 - protein, 266 aa, synthetic construct
  REGION 1..266: note = Description of Artificial Sequence: Synthetic polypeptide
MFVFLVLLPLVSSQCVVRFPNITNLCPFGEVFNATRFASVYAWNRKRISNCVADYSVLYNSASFSTFKCYGVSPTKLNDLCFTNVYADSFVIRGDEVRQIAPGQTGKIADYNYKLPDDFTGCVIAWNSNNLDSKVGGNYNYLYRLFRKSNLKPFERDISTEIYQAGSTPCNGVEGFNCYFPLQSYGFQPTNGVGYQPYRVVVLSFELLHAPATVCGPKGSPGSGSGSGYIPEAPRDGQAYVRKDGEWVLLSTFLGRSLEVLFQGPG

SEQ ID NO: 22 - RNA, 798 nt, synthetic construct
  misc_feature 1..798: note = Description of Artificial Sequence: Synthetic polynucleotide
  source 1..798: mol_type = other RNA
atgtttgtgtttcttgtgctgctgcctcttgtgtcttctcagtgtgtggtgagatttccaaatattacaaatctgtgtccatttggagaagtgtttaatgcaacaagatttgcatctgtgtatgcatggaatagaaaaagaatttctaattgtgtggctgattattctgtgctgtataatagtgcttctttttccacatttaaatgttatggagtgtctccaacaaaattaaatgatttatgttttacaaatgtgtatgctgattcttttgtgatcagaggtgatgaagtgagacagattgcccccggacagacaggaaaaattgctgattacaattacaaactgcctgatgattttacaggatgtgtgattgcttggaattctaataatttagattctaaagtgggaggaaattacaattatctgtacagactgtttagaaaatcaaatctgaaaccttttgaaagagatatttcaacagaaatttatcaggctggatcaacaccttgtaatggagtggaaggatttaattgttattttccattacagagctatggatttcagccaaccaatggtgtgggatatcagccatatagagtggtggtgctgtcttttgaactgctgcatgcacctgcaacagtgtgtggacctaaaggctcccccggctccggctccggatctggttatattcctgaagctccaagagatgggcaagcttacgttcgtaaagatggcgaatgggtattactttctacctttttaggccggtccctggaggtgctgttccagggccccggc

SEQ ID NO: 23 - RNA, 3819 nt, synthetic construct
  misc_feature 1..3819: note = Description of Artificial Sequence: Synthetic polynucleotide
  source 1..3819: mol_type = other RNA
atgtttgtgtttcttgtgctgctgcctcttgtgtcttctcagtgtgtgaatttgacaacaagaacacagctgccaccagcttatacaaattcttttaccagaggagtgtattatcctgataaagtgtttagatcttctgtgctgcacagcacacaggacctgtttctgccattttttagcaatgtgacatggtttcatgcaattcatgtgtctggaacaaatggaacaaaaagatttgataatcctgtgctgccttttaatgatggagtgtattttgcttcaacagaaaagtcaaatattattagaggatggatttttggaacaacactggattctaaaacacagtctctgctgattgtgaataatgcaacaaatgtggtgattaaagtgtgtgaatttcagttttgtaatgatccttttctgggagtgtattatcacaaaaataataaatcttggatggaatctgaatttagagtgtattcctctgcaaataattgtacatttgaatatgtgtctcagccttttctgatggatctggaaggaaaacagggcaattttaaaaatctgagagaatttgtgtttaaaaatattgatggatattttaaaatttattctaaacacacaccaattaatttagtgagagatctgcctcagggattttctgctctggaacctctggtggatctgccaattggcattaatattacaagatttcagacactgctggctctgcacagatcttatctgacacctggagattcttcttctggatggacagccggagctgcagcttattatgtgggctatctgcagccaagaacatttctgctgaaatataatgaaaatggaacaattacagatgctgtggattgtgctctggatcctctgtctgaaacaaaatgtacattaaaatcttttacagtggaaaaaggcatttatcagacatctaattttagagtgcagccaacagaatctattgtgagatttccaaatattacaaatctgtgtccatttggagaagtgtttaatgcaacaagatttgcatctgtgtatgcatggaatagaaaaagaatttctaattgtgtggctgattattctgtgctgtataatagtgcttctttttccacatttaaatgttatggagtgtctccaacaaaattaaatgatttatgttttacaaatgtgtatgctgattcttttgtgatcagaggtgatgaagtgagacagattgcccccggacagacaggaaaaattgctgattacaattacaaactgcctgatgattttacaggatgtgtgattgcttggaattctaataatttagattctaaagtgggaggaaattacaattatctgtacagactgtttagaaaatcaaatctgaaaccttttgaaagagatatttcaacagaaatttatcaggctggatcaacaccttgtaatggagtggaaggatttaattgttattttccattacagagctatggatttcagccaaccaatggtgtgggatatcagccatatagagtggtggtgctgtcttttgaactgctgcatgcacctgcaacagtgtgtggacctaaaaaatctacaaatttagtgaaaaataaatgtgtgaattttaattttaatggattaacaggaacaggagtgctgacagaatctaataaaaaatttctgccttttcagcagtttggcagagatattgcagataccacagatgcagtgagagatcctcagacattagaaattctggatattacaccttgttcttttgggggtgtgtctgtgattacacctggaacaaatacatctaatcaggtggctgtgctgtatcaggatgtgaattgtacagaagtgccagtggcaattcatgcagatcagctgacaccaacatggagagtgtattctacaggatctaatgtgtttcagacaagagcaggatgtctgattggagcagaacatgtgaataattcttatgaatgtgatattccaattggagcaggcatttgtgcatcttatcagacacagacaaattccccaaggagagcaagatctgtggcatctcagtctattattgcatacaccatgtctctgggagcagaaaattctgtggcatattctaataattctattgctattccaacaaattttaccatttctgtgacaacagaaattttacctgtgtctatgacaaaaacatctgtggattgtaccatgtacatttgtggagattctacagaatgttctaatctgctgctgcagtatggatctttttgtacacagctgaatagagctttaacaggaattgctgtggaacaggataaaaatacacaggaagtgtttgctcaggtgaaacagatttacaaaacaccaccaattaaagattttggaggatttaattttagccagattctgcctgatccttctaaaccttctaaaagatcttttattgaagatctgctgtttaataaagtgacactggcagatgcaggatttattaaacagtatggagattgcctgggtgatattgctgcaagagatctgatttgtgctcagaaatttaatggactgacagtgctgcctcctctgctgacagatgaaatgattgctcagtacacatctgctttactggctggaacaattacaagcggatggacatttggagctggagctgctctgcagattccttttgcaatgcagatggcttacagatttaatggaattggagtgacacagaatgtgttatatgaaaatcagaaactgattgcaaatcagtttaattctgcaattggcaaaattcaggattctctgtcttctacagcttctgctctgggaaaactgcaggatgtggtgaatcagaatgcacaggcactgaatactctggtgaaacagctgtctagcaattttggggcaatttcttctgtgctgaatgatattctgtctagactggatcctcctgaagctgaagtgcagattgatagactgatcacaggaagactgcagtctctgcagacttatgtgacacagcagctgattagagctgctgaaattagagcttctgctaatctggctgctacaaaaatgtctgaatgtgtgctgggacagtcaaaaagagtggatttttgtggaaaaggatatcatctgatgtcttttccacagtctgctccacatggagtggtgtttttacatgtgacatatgtgccagcacaggaaaagaattttaccacagcaccagcaatttgtcatgatggaaaagcacattttccaagagaaggagtgtttgtgtctaatggaacacattggtttgtgacacagagaaatttttatgaacctcagattattacaacagataatacatttgtgtcaggaaattgtgatgtggtgattggaattgtgaataatacagtgtatgatccactgcagccagaactggattcttttaaagaagaactggataaatattttaaaaatcacacatctcctgatgtggatttaggagatatttctggaatcaatgcatctgtggtgaatattcagaaagaaattgatagactgaatgaagtggccaaaaatctgaatgaatctctgattgatctgcaggaacttggaaaatatgaacagtacattaaatggccttggtacatttggcttggatttattgcaggattaattgcaattgtgatggtgacaattatgttatgttgtatgacatcatgttgttcttgtttaaaaggatgttgttcttgtggaagctgttgtaaatttgatgaagatgattctgaacctgtgttaaaaggagtgaaattgcattacaca

SEQ ID NO: 24 - RNA, 3819 nt, synthetic construct
  misc_feature 1..3819: note = Description of Artificial Sequence: Synthetic polynucleotide
  source 1..3819: mol_type = other RNA
atgttcgtgttcctggtgctgctgcctctggtgtccagccagtgtgtgaacctgaccaccagaacacagctgcctccagcctacaccaacagctttaccagaggcgtgtactaccccgacaaggtgttcagatccagcgtgctgcactctacccaggacctgttcctgcctttcttcagcaacgtgacctggttccacgccatccacgtgtccggcaccaatggcaccaagagattcgacaaccccgtgctgcccttcaacgacggggtgtactttgccagcaccgagaagtccaacatcatcagaggctggatcttcggcaccacactggacagcaagacccagagcctgctgatcgtgaacaacgccaccaacgtggtcatcaaagtgtgcgagttccagttctgcaacgaccccttcctgggcgtctactaccacaagaacaacaagagctggatggaaagcgagttccgggtgtacagcagcgccaacaactgcaccttcgagtacgtgtcccagcctttcctgatggacctggaaggcaagcagggcaacttcaagaacctgcgcgagttcgtgtttaagaacatcgacggctacttcaagatctacagcaagcacacccctatcaacctcgtgcgggatctgcctcagggcttctctgctctggaacccctggtggatctgcccatcggcatcaacatcacccggtttcagacactgctggccctgcacagaagctacctgacacctggcgatagcagcagcggatggacagctggtgccgccgcttactatgtgggctacctgcagcctagaaccttcctgctgaagtacaacgagaacggcaccatcaccgacgccgtggattgtgctctggatcctctgagcgagacaaagtgcaccctgaagtccttcaccgtggaaaagggcatctaccagaccagcaacttccgggtgcagcccaccgaatccatcgtgcggttccccaatatcaccaatctgtgccccttcggcgaggtgttcaatgccaccagattcgcctctgtgtacgcctggaaccggaagcggatcagcaattgcgtggccgactactccgtgctgtacaactccgccagcttcagcaccttcaagtgctacggcgtgtcccctaccaagctgaacgacctgtgcttcacaaacgtgtacgccgacagcttcgtgatccggggagatgaagtgcggcagattgcccctggacagacaggcaagatcgccgactacaactacaagctgcccgacgacttcaccggctgtgtgattgcctggaacagcaacaacctggactccaaagtcggcggcaactacaattacctgtaccggctgttccggaagtccaatctgaagcccttcgagcgggacatctccaccgagatctatcaggccggcagcaccccttgtaacggcgtggaaggcttcaactgctacttcccactgcagtcctacggctttcagcccacaaatggcgtgggctatcagccctacagagtggtggtgctgagcttcgaactgctgcatgcccctgccacagtgtgcggccctaagaaaagcaccaatctcgtgaagaacaaatgcgtgaacttcaacttcaacggcctgaccggcaccggcgtgctgacagagagcaacaagaagttcctgccattccagcagtttggccgggatatcgccgataccacagacgccgttagagatccccagacactggaaatcctggacatcaccccttgcagcttcggcggagtgtctgtgatcacccctggcaccaacaccagcaatcaggtggcagtgctgtaccaggacgtgaactgtaccgaagtgcccgtggccattcacgccgatcagctgacacctacatggcgggtgtactccaccggcagcaatgtgtttcagaccagagccggctgtctgatcggagccgagcacgtgaacaatagctacgagtgcgacatccccatcggcgctggaatctgcgccagctaccagacacagacaaacagccctcggagagccagaagcgtggccagccagagcatcattgcctacacaatgtctctgggcgccgagaacagcgtggcctactccaacaactctatcgctatccccaccaacttcaccatcagcgtgaccacagagatcctgcctgtgtccatgaccaagaccagcgtggactgcaccatgtacatctgcggcgattccaccgagtgctccaacctgctgctgcagtacggcagcttctgcacccagctgaatagagccctgacagggatcgccgtggaacaggacaagaacacccaagaggtgttcgcccaagtgaagcagatctacaagacccctcctatcaaggacttcggcggcttcaatttcagccagattctgcccgatcctagcaagcccagcaagcggagcttcatcgaggacctgctgttcaacaaagtgacactggccgacgccggcttcatcaagcagtatggcgattgtctgggcgacattgccgccagggatctgatttgcgcccagaagtttaacggactgacagtgctgcctcctctgctgaccgatgagatgatcgcccagtacacatctgccctgctggccggcacaatcacaagcggctggacatttggagcaggcgccgctctgcagatcccctttgctatgcagatggcctaccggttcaacggcatcggagtgacccagaatgtgctgtacgagaaccagaagctgatcgccaaccagttcaacagcgccatcggcaagatccaggacagcctgagcagcacagcaagcgccctgggaaagctgcaggacgtggtcaaccagaatgcccaggcactgaacaccctggtcaagcagctgtcctccaacttcggcgccatcagctctgtgctgaacgatatcctgagcagactggaccctcctgaggccgaggtgcagatcgacagactgatcacaggcagactgcagagcctccagacatacgtgacccagcagctgatcagagccgccgagattagagcctctgccaatctggccgccaccaagatgtctgagtgtgtgctgggccagagcaagagagtggacttttgcggcaagggctaccacctgatgagcttccctcagtctgcccctcacggcgtggtgtttctgcacgtgacatatgtgcccgctcaagagaagaatttcaccaccgctccagccatctgccacgacggcaaagcccactttcctagagaaggcgtgttcgtgtccaacggcacccattggttcgtgacacagcggaacttctacgagccccagatcatcaccaccgacaacaccttcgtgtctggcaactgcgacgtcgtgatcggcattgtgaacaataccgtgtacgaccctctgcagcccgagctggacagcttcaaagaggaactggacaagtactttaagaaccacacaagccccgacgtggacctgggcgatatcagcggaatcaatgccagcgtcgtgaacatccagaaagagatcgaccggctgaacgaggtggccaagaatctgaacgagagcctgatcgacctgcaagaactggggaagtacgagcagtacatcaagtggccctggtacatctggctgggctttatcgccggactgattgccatcgtgatggtcacaatcatgctgtgttgcatgaccagctgctgtagctgcctgaagggctgttgtagctgtggcagctgctgcaagttcgacgaggacgattctgagcccgtgctgaagggcgtgaaactgcactacaca

SEQ ID NO: 25 - protein, 41 aa, synthetic construct
  REGION 1..41: note = Description of Artificial Sequence: Synthetic polypeptide
GSGYIPEAPRDGQAYVRKDGEWVLLSTFLGRSLEVLFQGPG

SEQ ID NO: 26 - RNA, 123 nt, synthetic construct
  misc_feature 1..123: note = Description of Artificial Sequence: Synthetic polynucleotide
  source 1..123: mol_type = other RNA
ggatctggttatattcctgaagctccaagagatgggcaagcttacgttcgtaaagatggcgaatgggtattactttctacctttttaggccggtccctggaggtgctgttccagggccccggc

SEQ ID NO: 27 - RNA, 47 nt, synthetic construct
  misc_feature 1..47: note = Description of Artificial Sequence: Synthetic oligonucleotide
  source 1..47: mol_type = other RNA
aactagtattcttctggtccccacagactcagagagaacccgccacc

SEQ ID NO: 28 - RNA, 4282 nt, synthetic construct
  misc_feature 1..4282: note = Description of Artificial Sequence: Synthetic polynucleotide
  source 1..4282: mol_type = other RNA
gggcgaactagtattcttctggtccccacagactcagagagaacccgccaccatgtttgtgtttcttgtgctgctgcctcttgtgtcttctcagtgtgtgaatttgacaacaagaacacagctgccaccagcttatacaaattcttttaccagaggagtgtattatcctgataaagtgtttagatcttctgtgctgcacagcacacaggacctgtttctgccattttttagcaatgtgacatggtttcatgcaattcatgtgtctggaacaaatggaacaaaaagatttgataatcctgtgctgccttttaatgatggagtgtattttgcttcaacagaaaagtcaaatattattagaggatggatttttggaacaacactggattctaaaacacagtctctgctgattgtgaataatgcaacaaatgtggtgattaaagtgtgtgaatttcagttttgtaatgatccttttctgggagtgtattatcacaaaaataataaatcttggatggaatctgaatttagagtgtattcctctgcaaataattgtacatttgaatatgtgtctcagccttttctgatggatctggaaggaaaacagggcaattttaaaaatctgagagaatttgtgtttaaaaatattgatggatattttaaaatttattctaaacacacaccaattaatttagtgagagatctgcctcagggattttctgctctggaacctctggtggatctgccaattggcattaatattacaagatttcagacactgctggctctgcacagatcttatctgacacctggagattcttcttctggatggacagccggagctgcagcttattatgtgggctatctgcagccaagaacatttctgctgaaatataatgaaaatggaacaattacagatgctgtggattgtgctctggatcctctgtctgaaacaaaatgtacattaaaatcttttacagtggaaaaaggcatttatcagacatctaattttagagtgcagccaacagaatctattgtgagatttccaaatattacaaatctgtgtccatttggagaagtgtttaatgcaacaagatttgcatctgtgtatgcatggaatagaaaaagaatttctaattgtgtggctgattattctgtgctgtataatagtgcttctttttccacatttaaatgttatggagtgtctccaacaaaattaaatgatttatgttttacaaatgtgtatgctgattcttttgtgatcagaggtgatgaagtgagacagattgcccccggacagacaggaaaaattgctgattacaattacaaactgcctgatgattttacaggatgtgtgattgcttggaattctaataatttagattctaaagtgggaggaaattacaattatctgtacagactgtttagaaaatcaaatctgaaaccttttgaaagagatatttcaacagaaatttatcaggctggatcaacaccttgtaatggagtggaaggatttaattgttattttccattacagagctatggatttcagccaaccaatggtgtgggatatcagccatatagagtggtggtgctgtcttttgaactgctgcatgcacctgcaacagtgtgtggacctaaaaaatctacaaatttagtgaaaaataaatgtgtgaattttaattttaatggattaacaggaacaggagtgctgacagaatctaataaaaaatttctgccttttcagcagtttggcagagatattgcagataccacagatgcagtgagagatcctcagacattagaaattctggatattacaccttgttcttttgggggtgtgtctgtgattacacctggaacaaatacatctaatcaggtggctgtgctgtatcaggatgtgaattgtacagaagtgccagtggcaattcatgcagatcagctgacaccaacatggagagtgtattctacaggatctaatgtgtttcagacaagagcaggatgtctgattggagcagaacatgtgaataattcttatgaatgtgatattccaattggagcaggcatttgtgcatcttatcagacacagacaaattccccaaggagagcaagatctgtggcatctcagtctattattgcatacaccatgtctctgggagcagaaaattctgtggcatattctaataattctattgctattccaacaaattttaccatttctgtgacaacagaaattttacctgtgtctatgacaaaaacatctgtggattgtaccatgtacatttgtggagattctacagaatgttctaatctgctgctgcagtatggatctttttgtacacagctgaatagagctttaacaggaattgctgtggaacaggataaaaatacacaggaagtgtttgctcaggtgaaacagatttacaaaacaccaccaattaaagattttggaggatttaattttagccagattctgcctgatccttctaaaccttctaaaagatcttttattgaagatctgctgtttaataaagtgacactggcagatgcaggatttattaaacagtatggagattgcctgggtgatattgctgcaagagatctgatttgtgctcagaaatttaatggactgacagtgctgcctcctctgctgacagatgaaatgattgctcagtacacatctgctttactggctggaacaattacaagcggatggacatttggagctggagctgctctgcagattccttttgcaatgcagatggcttacagatttaatggaattggagtgacacagaatgtgttatatgaaaatcagaaactgattgcaaatcagtttaattctgcaattggcaaaattcaggattctctgtcttctacagcttctgctctgggaaaactgcaggatgtggtgaatcagaatgcacaggcactgaatactctggtgaaacagctgtctagcaattttggggcaatttcttctgtgctgaatgatattctgtctagactggatcctcctgaagctgaagtgcagattgatagactgatcacaggaagactgcagtctctgcagacttatgtgacacagcagctgattagagctgctgaaattagagcttctgctaatctggctgctacaaaaatgtctgaatgtgtgctgggacagtcaaaaagagtggatttttgtggaaaaggatatcatctgatgtcttttccacagtctgctccacatggagtggtgtttttacatgtgacatatgtgccagcacaggaaaagaattttaccacagcaccagcaatttgtcatgatggaaaagcacattttccaagagaaggagtgtttgtgtctaatggaacacattggtttgtgacacagagaaatttttatgaacctcagattattacaacagataatacatttgtgtcaggaaattgtgatgtggtgattggaattgtgaataatacagtgtatgatccactgcagccagaactggattcttttaaagaagaactggataaatattttaaaaatcacacatctcctgatgtggatttaggagatatttctggaatcaatgcatctgtggtgaatattcagaaagaaattgatagactgaatgaagtggccaaaaatctgaatgaatctctgattgatctgcaggaacttggaaaatatgaacagtacattaaatggccttggtacatttggcttggatttattgcaggattaattgcaattgtgatggtgacaattatgttatgttgtatgacatcatgttgttcttgtttaaaaggatgttgttcttgtggaagctgttgtaaatttgatgaagatgattctgaacctgtgttaaaaggagtgaaattgcattacacatgatgactcgagctggtactgcatgcacgcaatgctagctgcccctttcccgtcctgggtaccccgagtctcccccgacctcgggtcccaggtatgctcccacctccacctgccccactcaccacctctgctagttccagacacctcccaagcacgcagcaatgcagctcaaaacgcttagcctagccacacccccacgggaaacagcagtgattaacctttagcaataaacgaaagtttaactaagctatactaaccccagggttggtcaatttcgtgccagccacaccctggagctagcaaaaaaaaaaaaaaaaaaaaaaaaaaaaaagcatatgactaaaaaaaaaaaaaaaaaaaaaaaaaaaaaaaaaaaaaaaaaaaaaaaaaaaaaaaaaaaaaaaaaaaaaa

SEQ ID NO: 29 - RNA, 4282 nt, synthetic construct
  misc_feature 1..4282: note = Description of Artificial Sequence: Synthetic polynucleotide
  source 1..4282: mol_type = other RNA
gggcgaactagtattcttctggtccccacagactcagagagaacccgccaccatgttcgtgttcctggtgctgctgcctctggtgtccagccagtgtgtgaacctgaccaccagaacacagctgcctccagcctacaccaacagctttaccagaggcgtgtactaccccgacaaggtgttcagatccagcgtgctgcactctacccaggacctgttcctgcctttcttcagcaacgtgacctggttccacgccatccacgtgtccggcaccaatggcaccaagagattcgacaaccccgtgctgcccttcaacgacggggtgtactttgccagcaccgagaagtccaacatcatcagaggctggatcttcggcaccacactggacagcaagacccagagcctgctgatcgtgaacaacgccaccaacgtggtcatcaaagtgtgcgagttccagttctgcaacgaccccttcctgggcgtctactaccacaagaacaacaagagctggatggaaagcgagttccgggtgtacagcagcgccaacaactgcaccttcgagtacgtgtcccagcctttcctgatggacctggaaggcaagcagggcaacttcaagaacctgcgcgagttcgtgtttaagaacatcgacggctacttcaagatctacagcaagcacacccctatcaacctcgtgcgggatctgcctcagggcttctctgctctggaacccctggtggatctgcccatcggcatcaacatcacccggtttcagacactgctggccctgcacagaagctacctgacacctggcgatagcagcagcggatggacagctggtgccgccgcttactatgtgggctacctgcagcctagaaccttcctgctgaagtacaacgagaacggcaccatcaccgacgccgtggattgtgctctggatcctctgagcgagacaaagtgcaccctgaagtccttcaccgtggaaaagggcatctaccagaccagcaacttccgggtgcagcccaccgaatccatcgtgcggttccccaatatcaccaatctgtgccccttcggcgaggtgttcaatgccaccagattcgcctctgtgtacgcctggaaccggaagcggatcagcaattgcgtggccgactactccgtgctgtacaactccgccagcttcagcaccttcaagtgctacggcgtgtcccctaccaagctgaacgacctgtgcttcacaaacgtgtacgccgacagcttcgtgatccggggagatgaagtgcggcagattgcccctggacagacaggcaagatcgccgactacaactacaagctgcccgacgacttcaccggctgtgtgattgcctggaacagcaacaacctggactccaaagtcggcggcaactacaattacctgtaccggctgttccggaagtccaatctgaagcccttcgagcgggacatctccaccgagatctatcaggccggcagcaccccttgtaacggcgtggaaggcttcaactgctacttcccactgcagtcctacggctttcagcccacaaatggcgtgggctatcagccctacagagtggtggtgctgagcttcgaactgctgcatgcccctgccacagtgtgcggccctaagaaaagcaccaatctcgtgaagaacaaatgcgtgaacttcaacttcaacggcctgaccggcaccggcgtgctgacagagagcaacaagaagttcctgccattccagcagtttggccgggatatcgccgataccacagacgccgttagagatccccagacactggaaatcctggacatcaccccttgcagcttcggcggagtgtctgtgatcacccctggcaccaacaccagcaatcaggtggcagtgctgtaccaggacgtgaactgtaccgaagtgcccgtggccattcacgccgatcagctgacacctacatggcgggtgtactccaccggcagcaatgtgtttcagaccagagccggctgtctgatcggagccgagcacgtgaacaatagctacgagtgcgacatccccatcggcgctggaatctgcgccagctaccagacacagacaaacagccctcggagagccagaagcgtggccagccagagcatcattgcctacacaatgtctctgggcgccgagaacagcgtggcctactccaacaactctatcgctatccccaccaacttcaccatcagcgtgaccacagagatcctgcctgtgtccatgaccaagaccagcgtggactgcaccatgtacatctgcggcgattccaccgagtgctccaacctgctgctgcagtacggcagcttctgcacccagctgaatagagccctgacagggatcgccgtggaacaggacaagaacacccaagaggtgttcgcccaagtgaagcagatctacaagacccctcctatcaaggacttcggcggcttcaatttcagccagattctgcccgatcctagcaagcccagcaagcggagcttcatcgaggacctgctgttcaacaaagtgacactggccgacgccggcttcatcaagcagtatggcgattgtctgggcgacattgccgccagggatctgatttgcgcccagaagtttaacggactgacagtgctgcctcctctgctgaccgatgagatgatcgcccagtacacatctgccctgctggccggcacaatcacaagcggctggacatttggagcaggcgccgctctgcagatcccctttgctatgcagatggcctaccggttcaacggcatcggagtgacccagaatgtgctgtacgagaaccagaagctgatcgccaaccagttcaacagcgccatcggcaagatccaggacagcctgagcagcacagcaagcgccctgggaaagctgcaggacgtggtcaaccagaatgcccaggcactgaacaccctggtcaagcagctgtcctccaacttcggcgccatcagctctgtgctgaacgatatcctgagcagactggaccctcctgaggccgaggtgcagatcgacagactgatcacaggcagactgcagagcctccagacatacgtgacccagcagctgatcagagccgccgagattagagcctctgccaatctggccgccaccaagatgtctgagtgtgtgctgggccagagcaagagagtggacttttgcggcaagggctaccacctgatgagcttccctcagtctgcccctcacggcgtggtgtttctgcacgtgacatatgtgcccgctcaagagaagaatttcaccaccgctccagccatctgccacgacggcaaagcccactttcctagagaaggcgtgttcgtgtccaacggcacccattggttcgtgacacagcggaacttctacgagccccagatcatcaccaccgacaacaccttcgtgtctggcaactgcgacgtcgtgatcggcattgtgaacaataccgtgtacgaccctctgcagcccgagctggacagcttcaaagaggaactggacaagtactttaagaaccacacaagccccgacgtggacctgggcgatatcagcggaatcaatgccagcgtcgtgaacatccagaaagagatcgaccggctgaacgaggtggccaagaatctgaacgagagcctgatcgacctgcaagaactggggaagtacgagcagtacatcaagtggccctggtacatctggctgggctttatcgccggactgattgccatcgtgatggtcacaatcatgctgtgttgcatgaccagctgctgtagctgcctgaagggctgttgtagctgtggcagctgctgcaagttcgacgaggacgattctgagcccgtgctgaagggcgtgaaactgcactacacatgatgactcgagctggtactgcatgcacgcaatgctagctgcccctttcccgtcctgggtaccccgagtctcccccgacctcgggtcccaggtatgctcccacctccacctgccccactcaccacctctgctagttccagacacctcccaagcacgcagcaatgcagctcaaaacgcttagcctagccacacccccacgggaaacagcagtgattaacctttagcaataaacgaaagtttaactaagctatactaaccccagggttggtcaatttcgtgccagccacaccctggagctagcaaaaaaaaaaaaaaaaaaaaaaaaaaaaaagcatatgactaaaaaaaaaaaaaaaaaaaaaaaaaaaaaaaaaaaaaaaaaaaaaaaaaaaaaaaaaaaaaaaaaaaaaa

SEQ ID NO: 30 - RNA, 1261 nt, synthetic construct
  misc_feature 1..1261: note = Description of Artificial Sequence: Synthetic polynucleotide
  source 1..1261: mol_type = other RNA
gggcgaactagtattcttctggtccccacagactcagagagaacccgccaccatgtttgtgtttcttgtgctgctgcctcttgtgtcttctcagtgtgtggtgagatttccaaatattacaaatctgtgtccatttggagaagtgtttaatgcaacaagatttgcatctgtgtatgcatggaatagaaaaagaatttctaattgtgtggctgattattctgtgctgtataatagtgcttctttttccacatttaaatgttatggagtgtctccaacaaaattaaatgatttatgttttacaaatgtgtatgctgattcttttgtgatcagaggtgatgaagtgagacagattgcccccggacagacaggaaaaattgctgattacaattacaaactgcctgatgattttacaggatgtgtgattgcttggaattctaataatttagattctaaagtgggaggaaattacaattatctgtacagactgtttagaaaatcaaatctgaaaccttttgaaagagatatttcaacagaaatttatcaggctggatcaacaccttgtaatggagtggaaggatttaattgttattttccattacagagctatggatttcagccaaccaatggtgtgggatatcagccatatagagtggtggtgctgtcttttgaactgctgcatgcacctgcaacagtgtgtggacctaaaggctcccccggctccggctccggatctggttatattcctgaagctccaagagatgggcaagcttacgttcgtaaagatggcgaatgggtattactttctacctttttaggccggtccctggaggtgctgttccagggccccggctgatgactcgagctggtactgcatgcacgcaatgctagctgcccctttcccgtcctgggtaccccgagtctcccccgacctcgggtcccaggtatgctcccacctccacctgccccactcaccacctctgctagttccagacacctcccaagcacgcagcaatgcagctcaaaacgcttagcctagccacacccccacgggaaacagcagtgattaacctttagcaataaacgaaagtttaactaagctatactaaccccagggttggtcaatttcgtgccagccacaccctggagctagcaaaaaaaaaaaaaaaaaaaaaaaaaaaaaagcatatgactaaaaaaaaaaaaaaaaaaaaaaaaaaaaaaaaaaaaaaaaaaaaaaaaaaaaaaaaaaaaaaaaaaaaaa

SEQ ID NO: 31 - RNA, 4283 nt, synthetic construct
  misc_feature 1..4283: note = Description of Artificial Sequence: Synthetic polynucleotide
  source 1..4283: mol_type = other RNA
agaataaactagtattcttctggtccccacagactcagagagaacccgccaccatgtttgtgtttcttgtgctgctgcctcttgtgtcttctcagtgtgtgaatttgacaacaagaacacagctgccaccagcttatacaaattcttttaccagaggagtgtattatcctgataaagtgtttagatcttctgtgctgcacagcacacaggacctgtttctgccattttttagcaatgtgacatggtttcatgcaattcatgtgtctggaacaaatggaacaaaaagatttgataatcctgtgctgccttttaatgatggagtgtattttgcttcaacagaaaagtcaaatattattagaggatggatttttggaacaacactggattctaaaacacagtctctgctgattgtgaataatgcaacaaatgtggtgattaaagtgtgtgaatttcagttttgtaatgatccttttctgggagtgtattatcacaaaaataataaatcttggatggaatctgaatttagagtgtattcctctgcaaataattgtacatttgaatatgtgtctcagccttttctgatggatctggaaggaaaacagggcaattttaaaaatctgagagaatttgtgtttaaaaatattgatggatattttaaaatttattctaaacacacaccaattaatttagtgagagatctgcctcagggattttctgctctggaacctctggtggatctgccaattggcattaatattacaagatttcagacactgctggctctgcacagatcttatctgacacctggagattcttcttctggatggacagccggagctgcagcttattatgtgggctatctgcagccaagaacatttctgctgaaatataatgaaaatggaacaattacagatgctgtggattgtgctctggatcctctgtctgaaacaaaatgtacattaaaatcttttacagtggaaaaaggcatttatcagacatctaattttagagtgcagccaacagaatctattgtgagatttccaaatattacaaatctgtgtccatttggagaagtgtttaatgcaacaagatttgcatctgtgtatgcatggaatagaaaaagaatttctaattgtgtggctgattattctgtgctgtataatagtgcttctttttccacatttaaatgttatggagtgtctccaacaaaattaaatgatttatgttttacaaatgtgtatgctgattcttttgtgatcagaggtgatgaagtgagacagattgcccccggacagacaggaaaaattgctgattacaattacaaactgcctgatgattttacaggatgtgtgattgcttggaattctaataatttagattctaaagtgggaggaaattacaattatctgtacagactgtttagaaaatcaaatctgaaaccttttgaaagagatatttcaacagaaatttatcaggctggatcaacaccttgtaatggagtggaaggatttaattgttattttccattacagagctatggatttcagccaaccaatggtgtgggatatcagccatatagagtggtggtgctgtcttttgaactgctgcatgcacctgcaacagtgtgtggacctaaaaaatctacaaatttagtgaaaaataaatgtgtgaattttaattttaatggattaacaggaacaggagtgctgacagaatctaataaaaaatttctgccttttcagcagtttggcagagatattgcagataccacagatgcagtgagagatcctcagacattagaaattctggatattacaccttgttcttttgggggtgtgtctgtgattacacctggaacaaatacatctaatcaggtggctgtgctgtatcaggatgtgaattgtacagaagtgccagtggcaattcatgcagatcagctgacaccaacatggagagtgtattctacaggatctaatgtgtttcagacaagagcaggatgtctgattggagcagaacatgtgaataattcttatgaatgtgatattccaattggagcaggcatttgtgcatcttatcagacacagacaaattccccaaggagagcaagatctgtggcatctcagtctattattgcatacaccatgtctctgggagcagaaaattctgtggcatattctaataattctattgctattccaacaaattttaccatttctgtgacaacagaaattttacctgtgtctatgacaaaaacatctgtggattgtaccatgtacatttgtggagattctacagaatgttctaatctgctgctgcagtatggatctttttgtacacagctgaatagagctttaacaggaattgctgtggaacaggataaaaatacacaggaagtgtttgctcaggtgaaacagatttacaaaacaccaccaattaaagattttggaggatttaattttagccagattctgcctgatccttctaaaccttctaaaagatcttttattgaagatctgctgtttaataaagtgacactggcagatgcaggatttattaaacagtatggagattgcctgggtgatattgctgcaagagatctgatttgtgctcagaaatttaatggactgacagtgctgcctcctctgctgacagatgaaatgattgctcagtacacatctgctttactggctggaacaattacaagcggatggacatttggagctggagctgctctgcagattccttttgcaatgcagatggcttacagatttaatggaattggagtgacacagaatgtgttatatgaaaatcagaaactgattgcaaatcagtttaattctgcaattggcaaaattcaggattctctgtcttctacagcttctgctctgggaaaactgcaggatgtggtgaatcagaatgcacaggcactgaatactctggtgaaacagctgtctagcaattttggggcaatttcttctgtgctgaatgatattctgtctagactggatcctcctgaagctgaagtgcagattgatagactgatcacaggaagactgcagtctctgcagacttatgtgacacagcagctgattagagctgctgaaattagagcttctgctaatctggctgctacaaaaatgtctgaatgtgtgctgggacagtcaaaaagagtggatttttgtggaaaaggatatcatctgatgtcttttccacagtctgctccacatggagtggtgtttttacatgtgacatatgtgccagcacaggaaaagaattttaccacagcaccagcaatttgtcatgatggaaaagcacattttccaagagaaggagtgtttgtgtctaatggaacacattggtttgtgacacagagaaatttttatgaacctcagattattacaacagataatacatttgtgtcaggaaattgtgatgtggtgattggaattgtgaataatacagtgtatgatccactgcagccagaactggattcttttaaagaagaactggataaatattttaaaaatcacacatctcctgatgtggatttaggagatatttctggaatcaatgcatctgtggtgaatattcagaaagaaattgatagactgaatgaagtggccaaaaatctgaatgaatctctgattgatctgcaggaacttggaaaatatgaacagtacattaaatggccttggtacatttggcttggatttattgcaggattaattgcaattgtgatggtgacaattatgttatgttgtatgacatcatgttgttcttgtttaaaaggatgttgttcttgtggaagctgttgtaaatttgatgaagatgattctgaacctgtgttaaaaggagtgaaattgcattacacatgatgactcgagctggtactgcatgcacgcaatgctagctgcccctttcccgtcctgggtaccccgagtctcccccgacctcgggtcccaggtatgctcccacctccacctgccccactcaccacctctgctagttccagacacctcccaagcacgcagcaatgcagctcaaaacgcttagcctagccacacccccacgggaaacagcagtgattaacctttagcaataaacgaaagtttaactaagctatactaaccccagggttggtcaatttcgtgccagccacaccctggagctagcaaaaaaaaaaaaaaaaaaaaaaaaaaaaaagcatatgactaaaaaaaaaaaaaaaaaaaaaaaaaaaaaaaaaaaaaaaaaaaaaaaaaaaaaaaaaaaaaaaaaaaaaa

SEQ ID NO: 32 - RNA, 1262 nt, synthetic construct
  misc_feature 1..1262: note = Description of Artificial Sequence: Synthetic polynucleotide
  source 1..1262: mol_type = other RNA
agaataaactagtattcttctggtccccacagactcagagagaacccgccaccatgtttgtgtttcttgtgctgctgcctcttgtgtcttctcagtgtgtggtgagatttccaaatattacaaatctgtgtccatttggagaagtgtttaatgcaacaagatttgcatctgtgtatgcatggaatagaaaaagaatttctaattgtgtggctgattattctgtgctgtataatagtgcttctttttccacatttaaatgttatggagtgtctccaacaaaattaaatgatttatgttttacaaatgtgtatgctgattcttttgtgatcagaggtgatgaagtgagacagattgcccccggacagacaggaaaaattgctgattacaattacaaactgcctgatgattttacaggatgtgtgattgcttggaattctaataatttagattctaaagtgggaggaaattacaattatctgtacagactgtttagaaaatcaaatctgaaaccttttgaaagagatatttcaacagaaatttatcaggctggatcaacaccttgtaatggagtggaaggatttaattgttattttccattacagagctatggatttcagccaaccaatggtgtgggatatcagccatatagagtggtggtgctgtcttttgaactgctgcatgcacctgcaacagtgtgtggacctaaaggctcccccggctccggctccggatctggttatattcctgaagctccaagagatgggcaagcttacgttcgtaaagatggcgaatgggtattactttctacctttttaggccggtccctggaggtgctgttccagggccccggctgatgactcgagctggtactgcatgcacgcaatgctagctgcccctttcccgtcctgggtaccccgagtctcccccgacctcgggtcccaggtatgctcccacctccacctgccccactcaccacctctgctagttccagacacctcccaagcacgcagcaatgcagctcaaaacgcttagcctagccacacccccacgggaaacagcagtgattaacctttagcaataaacgaaagtttaactaagctatactaaccccagggttggtcaatttcgtgccagccacaccctggagctagcaaaaaaaaaaaaaaaaaaaaaaaaaaaaaagcatatgactaaaaaaaaaaaaaaaaaaaaaaaaaaaaaaaaaaaaaaaaaaaaaaaaaaaaaaaaaaaaaaaaaaaaaa

SEQ ID NO: 33 - RNA, 11917 nt, synthetic construct
  misc_feature 1..11917: note = Description of Artificial Sequence: Synthetic polynucleotide
  source 1..11917: mol_type = other RNA
gatgggcggcgcatgagagaagcccagaccaattacctacccaaaatggagaaagttcacgttgacatcgaggaagacagcccattcctcagagctttgcagcggagcttcccgcagtttgaggtagaagccaagcaggtcactgataatgaccatgctaatgccagagcgttttcgcatctggcttcaaaactgatcgaaacggaggtggacccatccgacacgatccttgacattggaagtgcgcccgcccgcagaatgtattctaagcacaagtatcattgtatctgtccgatgagatgtgcggaagatccggacagattgtataagtatgcaactaagctgaagaaaaactgtaaggaaataactgataaggaattggacaagaaaatgaaggagctcgccgccgtcatgagcgaccctgacctggaaactgagactatgtgcctccacgacgacgagtcgtgtcgctacgaagggcaagtcgctgtttaccaggatgtatacgcggttgacggaccgacaagtctctatcaccaagccaataagggagttagagtcgcctactggataggctttgacaccaccccttttatgtttaagaacttggctggagcatatccatcatactctaccaactgggccgacgaaaccgtgttaacggctcgtaacataggcctatgcagctctgacgttatggagcggtcacgtagagggatgtccattcttagaaagaagtatttgaaaccatccaacaatgttctattctctgttggctcgaccatctaccacgaaaagagggacttactgaggagctggcacctgccgtctgtatttcacttacgtggcaagcaaaattacacatgtcggtgtgagactatagttagttgcgacgggtacgtcgttaaaagaatagctatcagtccaggcctgtatgggaagccttcaggctatgctgctacgatgcaccgcgagggattcttgtgctgcaaagtgacagacacattgaacggggagagggtctcttttcccgtgtgcacgtatgtgccagctacattgtgtgaccaaatgactggcatactggcaacagatgtcagtgcggacgacgcgcaaaaactgctggttgggctcaaccagcgtatagtcgtcaacggtcgcacccagagaaacaccaataccatgaaaaattaccttttgcccgtagtggcccaggcatttgctaggtgggcaaaggaatataaggaagatcaagaagatgaaaggccactaggactacgagatagacagttagtcatggggtgttgttgggcttttagaaggcacaagataacatctatttataagcgcccggatacccaaaccatcatcaaagtgaacagcgatttccactcattcgtgctgcccaggataggcagtaacacattggagatcgggctgagaacaagaatcaggaaaatgttagaggagcacaaggagccgtcacctctcattaccgccgaggacgtacaagaagctaagtgcgcagccgatgaggctaaggaggtgcgtgaagccgaggagttgcgcgcagctctaccacctttggcagctgatgttgaggagcccactctggaagccgatgtcgacttgatgttacaagaggctggggccggctcagtggagacacctcgtggcttgataaaggttaccagctacgctggcgaggacaagatcggctcttacgctgtgctttctccgcaggctgtactcaagagtgaaaaattatcttgcatccaccctctcgctgaacaagtcatagtgataacacactctggccgaaaagggcgttatgccgtggaaccataccatggtaaagtagtggtgccagagggacatgcaatacccgtccaggactttcaagctctgagtgaaagtgccaccattgtgtacaacgaacgtgagttcgtaaacaggtacctgcaccatattgccacacatggaggagcgctgaacactgatgaagaatattacaaaactgtcaagcccagcgagcacgacggcgaatacctgtacgacatcgacaggaaacagtgcgtcaagaaagagctagtcactgggctagggctcacaggcgagctggtcgatcctcccttccatgaattcgcctacgagagtctgagaacacgaccagccgctccttaccaagtaccaaccataggggtgtatggcgtgccaggatcaggcaagtctggcatcattaaaagcgcagtcaccaaaaaagatctagtggtgagcgccaagaaagaaaactgtgcagaaattataagggacgtcaagaaaatgaaagggctggacgtcaatgccagaactgtggactcagtgctcttgaatggatgcaaacaccccgtagagaccctgtatattgacgaggcttttgcttgtcatgcaggtactctcagagcgctcatagccattataagacctaaaaaggcagtgctctgcggagatcccaaacagtgcggtttttttaacatgatgtgcctgaaagtgcattttaaccacgagatttgcacacaagtcttccacaaaagcatctctcgccgttgcactaaatctgtgacttcggtcgtctcaaccttgttttacgacaaaaaaatgagaacgacgaatccgaaagagactaagattgtgattgacactaccggcagtaccaaacctaagcaggacgatctcattctcacttgtttcagagggtgggtgaagcagttgcaaatagattacaaaggcaacgaaataatgacggcagctgcctctcaagggctgacccgtaaaggtgtgtatgccgttcggtacaaggtgaatgaaaatcctctgtacgcacccacctcagaacatgtgaacgtcctactgacccgcacggaggaccgcatcgtgtggaaaacactagccggcgacccatggataaaaacactgactgccaagtaccctgggaatttcactgccacgatagaggagtggcaagcagagcatgatgccatcatgaggcacatcttggagagaccggaccctaccgacgtcttccagaataaggcaaacgtgtgttgggccaaggctttagtgccggtgctgaagaccgctggcatagacatgaccactgaacaatggaacactgtggattattttgaaacggacaaagctcactcagcagagatagtattgaaccaactatgcgtgaggttctttggactcgatctggactccggtctattttctgcacccactgttccgttatccattaggaataatcactgggataactccccgtcgcctaacatgtacgggctgaataaagaagtggtccgtcagctctctcgcaggtacccacaactgcctcgggcagttgccactggtagagtctatgacatgaacactggtacactgcgcaattatgatccgcgcataaacctagtacctgtaaacagaagactgcctcatgctttagtcctccaccataatgaacacccacagagtgacttttcttcattcgtcagcaaattgaagggcagaactgtcctggtggtcggggaaaagttgtccgtcccaggcaaaatggttgactggttgtcagaccggcctgaggctaccttcagagctcggctggatttaggcatcccaggtgatgtgcccaaatatgacataatatttgttaatgtgaggaccccatataaataccatcactatcagcagtgtgaagaccatgccattaagctaagcatgttgaccaagaaagcatgtctgcatctgaatcccggcggaacctgtgtcagcataggttatggttacgctgacagggccagcgaaagcatcattggtgctatagcgcggcagttcaagttttcccgagtatgcaaaccgaaatcctcacttgaggagacggaagttctgtttgtattcattgggtacgatcgcaaggcccgtacgcacaatccttacaagctatcatcaaccttgaccaacatttatacaggttccagactccacgaagccggatgtgcaccctcatatcatgtggtgcgaggggatattgccacggccaccgaaggagtgattataaatgctgctaacagcaaaggacaacctggcggaggggtgtgcggagcgctgtataagaaattcccggaaagtttcgatttacagccgatcgaagtaggaaaagcgcgactggtcaaaggtgcagctaaacatatcattcatgccgtaggaccaaacttcaacaaagtttcggaggttgaaggtgacaaacagttggcagaggcttatgagtccatcgctaagattgtcaacgataacaattacaagtcagtagcgattccactgttgtccaccggcatcttttccgggaacaaagatcgactaacccaatcattgaaccatttgctgacagctttagacaccactgatgcagatgtagccatatactgcagggacaagaaatgggaaatgactctcaaggaagcagtggctaggagagaagcagtggaggagatatgcatatccgacgattcttcagtgacagaacctgatgcagagctggtgagggtgcatcccaagagttctttggctggaaggaagggctacagcacaagcgatggcaaaactttctcatatttggaagggaccaagtttcaccaggcggccaaggatatagcagaaattaatgccatgtggcccgttgcaacggaggccaatgagcaggtatgcatgtatatcctcggagaaagcatgagcagtattaggtcgaaatgccccgtcgaggagtcggaagcctccacaccacctagcacgctgccttgcttgtgcatccatgccatgactccagaaagagtacagcgcctaaaagcctcacgtccagaacaaattactgtgtgctcatcctttccattgccgaagtatagaatcactggtgtgcagaagatccaatgctcccagcctatattgttctcaccgaaagtgcctgcgtatattcatccaaggaagtatctcgtggaaacaccaccggtagacgagactccggagccatcggcagagaaccaatccacagaggggacacctgaacaaccaccacttataaccgaggatgagaccaggactagaacgcctgagccgatcatcatcgaagaagaagaagaagatagcataagtttgctgtcagatggcccgacccaccaggtgctgcaagtcgaggcagacattcacgggccgccctctgtatctagctcatcctggtccattcctcatgcatccgactttgatgtggacagtttatccatacttgacaccctggagggagctagcgtgaccagcggggcaacgtcagccgagactaactcttacttcgcaaagagtatggagtttctggcgcgaccggtgcctgcgcctcgaacagtattcaggaaccctccacatcccgctccgcgcacaagaacaccgtcacttgcacccagcagggcctgctccagaaccagcctagtttccaccccgccaggcgtgaatagggtgatcactagagaggagctcgaagcgcttaccccgtcacgcactcctagcaggtcggtctccagaaccagcctggtctccaacccgccaggcgtaaatagggtgattacaagagaggagtttgaggcgttcgtagcacaacaacaatgacggtttgatgcgggtgcatacatcttttcctccgacaccggtcaagggcatttacaacaaaaatcagtaaggcaaacggtgctatccgaagtggtgttggagaggaccgaattggagatttcgtatgccccgcgcctcgaccaagaaaaagaagaattactacgcaagaaattacagttaaatcccacacctgctaacagaagcagataccagtccaggaaggtggagaacatgaaagccataacagctagacgtattctgcaaggcctagggcattatttgaaggcagaaggaaaagtggagtgctaccgaaccctgcatcctgttcctttgtattcatctagtgtgaaccgtgccttttcaagccccaaggtcgcagtggaagcctgtaacgccatgttgaaagagaactttccgactgtggcttcttactgtattattccagagtacgatgcctatttggacatggttgacggagcttcatgctgcttagacactgccagtttttgccctgcaaagctgcgcagctttccaaagaaacactcctatttggaacccacaatacgatcggcagtgccttcagcgatccagaacacgctccagaacgtcctggcagctgccacaaaaagaaattgcaatgtcacgcaaatgagagaattgcccgtattggattcggcggcctttaatgtggaatgcttcaagaaatatgcgtgtaataatgaatattgggaaacgtttaaagaaaaccccatcaggcttactgaagaaaacgtggtaaattacattaccaaattaaaaggaccaaaagctgctgctctttttgcgaagacacataatttgaatatgttgcaggacataccaatggacaggtttgtaatggacttaaagagagacgtgaaagtgactccaggaacaaaacatactgaagaacggcccaaggtacaggtgatccaggctgccgatccgctagcaacagcgtatctgtgcggaatccaccgagagctggttaggagattaaatgcggtcctgcttccgaacattcatacactgtttgatatgtcggctgaagactttgacgctattatagccgagcacttccagcctggggattgtgttctggaaactgacatcgcgtcgtttgataaaagtgaggacgacgccatggctctgaccgcgttaatgattctggaagacttaggtgtggacgcagagctgttgacgctgattgaggcggctttcggcgaaatttcatcaatacatttgcccactaaaactaaatttaaattcggagccatgatgaaatctggaatgttcctcacactgtttgtgaacacagtcattaacattgtaatcgcaagcagagtgttgagagaacggctaaccggatcaccatgtgcagcattcattggagatgacaatatcgtgaaaggagtcaaatcggacaaattaatggcagacaggtgcgccacctggttgaatatggaagtcaagattatagatgctgtggtgggcgagaaagcgccttatttctgtggagggtttattttgtgtgactccgtgaccggcacagcgtgccgtgtggcagaccccctaaaaaggctgtttaagctaggcaaacctctggcagcagacgatgaacatgatgatgacaggagaagggcattgcatgaggagtcaacacgctggaaccgagtgggtattctttcagagctgtgcaaggcagtagaatcaaggtatgaaaccgtaggaacttccatcatagttatggccatgactactctagctagcagtgttaaatcattcagctacctgagaggggcccctataactctctacggctaacctgaatggactacgacatagtctagtccgccaagactagtatgtttgtgtttcttgtgctgctgcctcttgtgtcttctcagtgtgtgaatttgacaacaagaacacagctgccaccagcttatacaaattcttttaccagaggagtgtattatcctgataaagtgtttagatcttctgtgctgcacagcacacaggacctgtttctgccattttttagcaatgtgacatggtttcatgcaattcatgtgtctggaacaaatggaacaaaaagatttgataatcctgtgctgccttttaatgatggagtgtattttgcttcaacagaaaagtcaaatattattagaggatggatttttggaacaacactggattctaaaacacagtctctgctgattgtgaataatgcaacaaatgtggtgattaaagtgtgtgaatttcagttttgtaatgatccttttctgggagtgtattatcacaaaaataataaatcttggatggaatctgaatttagagtgtattcctctgcaaataattgtacatttgaatatgtgtctcagccttttctgatggatctggaaggaaaacagggcaattttaaaaatctgagagaatttgtgtttaaaaatattgatggatattttaaaatttattctaaacacacaccaattaatttagtgagagatctgcctcagggattttctgctctggaacctctggtggatctgccaattggcattaatattacaagatttcagacactgctggctctgcacagatcttatctgacacctggagattcttcttctggatggacagccggagctgcagcttattatgtgggctatctgcagccaagaacatttctgctgaaatataatgaaaatggaacaattacagatgctgtggattgtgctctggatcctctgtctgaaacaaaatgtacattaaaatcttttacagtggaaaaaggcatttatcagacatctaattttagagtgcagccaacagaatctattgtgagatttccaaatattacaaatctgtgtccatttggagaagtgtttaatgcaacaagatttgcatctgtgtatgcatggaatagaaaaagaatttctaattgtgtggctgattattctgtgctgtataatagtgcttctttttccacatttaaatgttatggagtgtctccaacaaaattaaatgatttatgttttacaaatgtgtatgctgattcttttgtgatcagaggtgatgaagtgagacagattgcccccggacagacaggaaaaattgctgattacaattacaaactgcctgatgattttacaggatgtgtgattgcttggaattctaataatttagattctaaagtgggaggaaattacaattatctgtacagactgtttagaaaatcaaatctgaaaccttttgaaagagatatttcaacagaaatttatcaggctggatcaacaccttgtaatggagtggaaggatttaattgttattttccattacagagctatggatttcagccaaccaatggtgtgggatatcagccatatagagtggtggtgctgtcttttgaactgctgcatgcacctgcaacagtgtgtggacctaaaaaatctacaaatttagtgaaaaataaatgtgtgaattttaattttaatggattaacaggaacaggagtgctgacagaatctaataaaaaatttctgccttttcagcagtttggcagagatattgcagataccacagatgcagtgagagatcctcagacattagaaattctggatattacaccttgttcttttgggggtgtgtctgtgattacacctggaacaaatacatctaatcaggtggctgtgctgtatcaggatgtgaattgtacagaagtgccagtggcaattcatgcagatcagctgacaccaacatggagagtgtattctacaggatctaatgtgtttcagacaagagcaggatgtctgattggagcagaacatgtgaataattcttatgaatgtgatattccaattggagcaggcatttgtgcatcttatcagacacagacaaattccccaaggagagcaagatctgtggcatctcagtctattattgcatacaccatgtctctgggagcagaaaattctgtggcatattctaataattctattgctattccaacaaattttaccatttctgtgacaacagaaattttacctgtgtctatgacaaaaacatctgtggattgtaccatgtacatttgtggagattctacagaatgttctaatctgctgctgcagtatggatctttttgtacacagctgaatagagctttaacaggaattgctgtggaacaggataaaaatacacaggaagtgtttgctcaggtgaaacagatttacaaaacaccaccaattaaagattttggaggatttaattttagccagattctgcctgatccttctaaaccttctaaaagatcttttattgaagatctgctgtttaataaagtgacactggcagatgcaggatttattaaacagtatggagattgcctgggtgatattgctgcaagagatctgatttgtgctcagaaatttaatggactgacagtgctgcctcctctgctgacagatgaaatgattgctcagtacacatctgctttactggctggaacaattacaagcggatggacatttggagctggagctgctctgcagattccttttgcaatgcagatggcttacagatttaatggaattggagtgacacagaatgtgttatatgaaaatcagaaactgattgcaaatcagtttaattctgcaattggcaaaattcaggattctctgtcttctacagcttctgctctgggaaaactgcaggatgtggtgaatcagaatgcacaggcactgaatactctggtgaaacagctgtctagcaattttggggcaatttcttctgtgctgaatgatattctgtctagactggatcctcctgaagctgaagtgcagattgatagactgatcacaggaagactgcagtctctgcagacttatgtgacacagcagctgattagagctgctgaaattagagcttctgctaatctggctgctacaaaaatgtctgaatgtgtgctgggacagtcaaaaagagtggatttttgtggaaaaggatatcatctgatgtcttttccacagtctgctccacatggagtggtgtttttacatgtgacatatgtgccagcacaggaaaagaattttaccacagcaccagcaatttgtcatgatggaaaagcacattttccaagagaaggagtgtttgtgtctaatggaacacattggtttgtgacacagagaaatttttatgaacctcagattattacaacagataatacatttgtgtcaggaaattgtgatgtggtgattggaattgtgaataatacagtgtatgatccactgcagccagaactggattcttttaaagaagaactggataaatattttaaaaatcacacatctcctgatgtggatttaggagatatttctggaatcaatgcatctgtggtgaatattcagaaagaaattgatagactgaatgaagtggccaaaaatctgaatgaatctctgattgatctgcaggaacttggaaaatatgaacagtacattaaatggccttggtacatttggcttggatttattgcaggattaattgcaattgtgatggtgacaattatgttatgttgtatgacatcatgttgttcttgtttaaaaggatgttgttcttgtggaagctgttgtaaatttgatgaagatgattctgaacctgtgttaaaaggagtgaaattgcattacacatgatgactcgagctggtactgcatgcacgcaatgctagctgcccctttcccgtcctgggtaccccgagtctcccccgacctcgggtcccaggtatgctcccacctccacctgccccactcaccacctctgctagttccagacacctcccaagcacgcagcaatgcagctcaaaacgcttagcctagccacacccccacgggaaacagcagtgattaacctttagcaataaacgaaagtttaactaagctatactaaccccagggttggtcaatttcgtgccagccacaccgcggccgcatgaatacagcagcaattggcaagctgcttacatagaactcgcggcgattggcatgccgccttaaaatttttattttattttttcttttcttttccgaatcggattttgtttttaatatttcaaaaaaaaaaaaaaaaaaaaaaaaaaaaaagcatatgactaaaaaaaaaaaaaaaaaaaaaaaaaaaaaaaaaaaaaaaaaaaaaaaaaaaaaaaaaaaaaaaaaaaaaa

SEQ ID NO: 34 - RNA, 11917 nt, synthetic construct
  misc_feature 1..11917: note = Description of Artificial Sequence: Synthetic polynucleotide
  source 1..11917: mol_type = other RNA
gatgggcggcgcatgagagaagcccagaccaattacctacccaaaatggagaaagttcacgttgacatcgaggaagacagcccattcctcagagctttgcagcggagcttcccgcagtttgaggtagaagccaagcaggtcactgataatgaccatgctaatgccagagcgttttcgcatctggcttcaaaactgatcgaaacggaggtggacccatccgacacgatccttgacattggaagtgcgcccgcccgcagaatgtattctaagcacaagtatcattgtatctgtccgatgagatgtgcggaagatccggacagattgtataagtatgcaactaagctgaagaaaaactgtaaggaaataactgataaggaattggacaagaaaatgaaggagctcgccgccgtcatgagcgaccctgacctggaaactgagactatgtgcctccacgacgacgagtcgtgtcgctacgaagggcaagtcgctgtttaccaggatgtatacgcggttgacggaccgacaagtctctatcaccaagccaataagggagttagagtcgcctactggataggctttgacaccaccccttttatgtttaagaacttggctggagcatatccatcatactctaccaactgggccgacgaaaccgtgttaacggctcgtaacataggcctatgcagctctgacgttatggagcggtcacgtagagggatgtccattcttagaaagaagtatttgaaaccatccaacaatgttctattctctgttggctcgaccatctaccacgaaaagagggacttactgaggagctggcacctgccgtctgtatttcacttacgtggcaagcaaaattacacatgtcggtgtgagactatagttagttgcgacgggtacgtcgttaaaagaatagctatcagtccaggcctgtatgggaagccttcaggctatgctgctacgatgcaccgcgagggattcttgtgctgcaaagtgacagacacattgaacggggagagggtctcttttcccgtgtgcacgtatgtgccagctacattgtgtgaccaaatgactggcatactggcaacagatgtcagtgcggacgacgcgcaaaaactgctggttgggctcaaccagcgtatagtcgtcaacggtcgcacccagagaaacaccaataccatgaaaaattaccttttgcccgtagtggcccaggcatttgctaggtgggcaaaggaatataaggaagatcaagaagatgaaaggccactaggactacgagatagacagttagtcatggggtgttgttgggcttttagaaggcacaagataacatctatttataagcgcccggatacccaaaccatcatcaaagtgaacagcgatttccactcattcgtgctgcccaggataggcagtaacacattggagatcgggctgagaacaagaatcaggaaaatgttagaggagcacaaggagccgtcacctctcattaccgccgaggacgtacaagaagctaagtgcgcagccgatgaggctaaggaggtgcgtgaagccgaggagttgcgcgcagctctaccacctttggcagctgatgttgaggagcccactctggaagccgatgtcgacttgatgttacaagaggctggggccggctcagtggagacacctcgtggcttgataaaggttaccagctacgctggcgaggacaagatcggctcttacgctgtgctttctccgcaggctgtactcaagagtgaaaaattatcttgcatccaccctctcgctgaacaagtcatagtgataacacactctggccgaaaagggcgttatgccgtggaaccataccatggtaaagtagtggtgccagagggacatgcaatacccgtccaggactttcaagctctgagtgaaagtgccaccattgtgtacaacgaacgtgagttcgtaaacaggtacctgcaccatattgccacacatggaggagcgctgaacactgatgaagaatattacaaaactgtcaagcccagcgagcacgacggcgaatacctgtacgacatcgacaggaaacagtgcgtcaagaaagagctagtcactgggctagggctcacaggcgagctggtcgatcctcccttccatgaattcgcctacgagagtctgagaacacgaccagccgctccttaccaagtaccaaccataggggtgtatggcgtgccaggatcaggcaagtctggcatcattaaaagcgcagtcaccaaaaaagatctagtggtgagcgccaagaaagaaaactgtgcagaaattataagggacgtcaagaaaatgaaagggctggacgtcaatgccagaactgtggactcagtgctcttgaatggatgcaaacaccccgtagagaccctgtatattgacgaggcttttgcttgtcatgcaggtactctcagagcgctcatagccattataagacctaaaaaggcagtgctctgcggagatcccaaacagtgcggtttttttaacatgatgtgcctgaaagtgcattttaaccacgagatttgcacacaagtcttccacaaaagcatctctcgccgttgcactaaatctgtgacttcggtcgtctcaaccttgttttacgacaaaaaaatgagaacgacgaatccgaaagagactaagattgtgattgacactaccggcagtaccaaacctaagcaggacgatctcattctcacttgtttcagagggtgggtgaagcagttgcaaatagattacaaaggcaacgaaataatgacggcagctgcctctcaagggctgacccgtaaaggtgtgtatgccgttcggtacaaggtgaatgaaaatcctctgtacgcacccacctcagaacatgtgaacgtcctactgacccgcacggaggaccgcatcgtgtggaaaacactagccggcgacccatggataaaaacactgactgccaagtaccctgggaatttcactgccacgatagaggagtggcaagcagagcatgatgccatcatgaggcacatcttggagagaccggaccctaccgacgtcttccagaataaggcaaacgtgtgttgggccaaggctttagtgccggtgctgaagaccgctggcatagacatgaccactgaacaatggaacactgtggattattttgaaacggacaaagctcactcagcagagatagtattgaaccaactatgcgtgaggttctttggactcgatctggactccggtctattttctgcacccactgttccgttatccattaggaataatcactgggataactccccgtcgcctaacatgtacgggctgaataaagaagtggtccgtcagctctctcgcaggtacccacaactgcctcgggcagttgccactggtagagtctatgacatgaacactggtacactgcgcaattatgatccgcgcataaacctagtacctgtaaacagaagactgcctcatgctttagtcctccaccataatgaacacccacagagtgacttttcttcattcgtcagcaaattgaagggcagaactgtcctggtggtcggggaaaagttgtccgtcccaggcaaaatggttgactggttgtcagaccggcctgaggctaccttcagagctcggctggatttaggcatcccaggtgatgtgcccaaatatgacataatatttgttaatgtgaggaccccatataaataccatcactatcagcagtgtgaagaccatgccattaagctaagcatgttgaccaagaaagcatgtctgcatctgaatcccggcggaacctgtgtcagcataggttatggttacgctgacagggccagcgaaagcatcattggtgctatagcgcggcagttcaagttttcccgagtatgcaaaccgaaatcctcacttgaggagacggaagttctgtttgtattcattgggtacgatcgcaaggcccgtacgcacaatccttacaagctatcatcaaccttgaccaacatttatacaggttccagactccacgaagccggatgtgcaccctcatatcatgtggtgcgaggggatattgccacggccaccgaaggagtgattataaatgctgctaacagcaaaggacaacctggcggaggggtgtgcggagcgctgtataagaaattcccggaaagtttcgatttacagccgatcgaagtaggaaaagcgcgactggtcaaaggtgcagctaaacatatcattcatgccgtaggaccaaacttcaacaaagtttcggaggttgaaggtgacaaacagttggcagaggcttatgagtccatcgctaagattgtcaacgataacaattacaagtcagtagcgattccactgttgtccaccggcatcttttccgggaacaaagatcgactaacccaatcattgaaccatttgctgacagctttagacaccactgatgcagatgtagccatatactgcagggacaagaaatgggaaatgactctcaaggaagcagtggctaggagagaagcagtggaggagatatgcatatccgacgattcttcagtgacagaacctgatgcagagctggtgagggtgcatcccaagagttctttggctggaaggaagggctacagcacaagcgatggcaaaactttctcatatttggaagggaccaagtttcaccaggcggccaaggatatagcagaaattaatgccatgtggcccgttgcaacggaggccaatgagcaggtatgcatgtatatcctcggagaaagcatgagcagtattaggtcgaaatgccccgtcgaggagtcggaagcctccacaccacctagcacgctgccttgcttgtgcatccatgccatgactccagaaagagtacagcgcctaaaagcctcacgtccagaacaaattactgtgtgctcatcctttccattgccgaagtatagaatcactggtgtgcagaagatccaatgctcccagcctatattgttctcaccgaaagtgcctgcgtatattcatccaaggaagtatctcgtggaaacaccaccggtagacgagactccggagccatcggcagagaaccaatccacagaggggacacctgaacaaccaccacttataaccgaggatgagaccaggactagaacgcctgagccgatcatcatcgaagaagaagaagaagatagcataagtttgctgtcagatggcccgacccaccaggtgctgcaagtcgaggcagacattcacgggccgccctctgtatctagctcatcctggtccattcctcatgcatccgactttgatgtggacagtttatccatacttgacaccctggagggagctagcgtgaccagcggggcaacgtcagccgagactaactcttacttcgcaaagagtatggagtttctggcgcgaccggtgcctgcgcctcgaacagtattcaggaaccctccacatcccgctccgcgcacaagaacaccgtcacttgcacccagcagggcctgctccagaaccagcctagtttccaccccgccaggcgtgaatagggtgatcactagagaggagctcgaagcgcttaccccgtcacgcactcctagcaggtcggtctccagaaccagcctggtctccaacccgccaggcgtaaatagggtgattacaagagaggagtttgaggcgttcgtagcacaacaacaatgacggtttgatgcgggtgcatacatcttttcctccgacaccggtcaagggcatttacaacaaaaatcagtaaggcaaacggtgctatccgaagtggtgttggagaggaccgaattggagatttcgtatgccccgcgcctcgaccaagaaaaagaagaattactacgcaagaaattacagttaaatcccacacctgctaacagaagcagataccagtccaggaaggtggagaacatgaaagccataacagctagacgtattctgcaaggcctagggcattatttgaaggcagaaggaaaagtggagtgctaccgaaccctgcatcctgttcctttgtattcatctagtgtgaaccgtgccttttcaagccccaaggtcgcagtggaagcctgtaacgccatgttgaaagagaactttccgactgtggcttcttactgtattattccagagtacgatgcctatttggacatggttgacggagcttcatgctgcttagacactgccagtttttgccctgcaaagctgcgcagctttccaaagaaacactcctatttggaacccacaatacgatcggcagtgccttcagcgatccagaacacgctccagaacgtcctggcagctgccacaaaaagaaattgcaatgtcacgcaaatgagagaattgcccgtattggattcggcggcctttaatgtggaatgcttcaagaaatatgcgtgtaataatgaatattgggaaacgtttaaagaaaaccccatcaggcttactgaagaaaacgtggtaaattacattaccaaattaaaaggaccaaaagctgctgctctttttgcgaagacacataatttgaatatgttgcaggacataccaatggacaggtttgtaatggacttaaagagagacgtgaaagtgactccaggaacaaaacatactgaagaacggcccaaggtacaggtgatccaggctgccgatccgctagcaacagcgtatctgtgcggaatccaccgagagctggttaggagattaaatgcggtcctgcttccgaacattcatacactgtttgatatgtcggctgaagactttgacgctattatagccgagcacttccagcctggggattgtgttctggaaactgacatcgcgtcgtttgataaaagtgaggacgacgccatggctctgaccgcgttaatgattctggaagacttaggtgtggacgcagagctgttgacgctgattgaggcggctttcggcgaaatttcatcaatacatttgcccactaaaactaaatttaaattcggagccatgatgaaatctggaatgttcctcacactgtttgtgaacacagtcattaacattgtaatcgcaagcagagtgttgagagaacggctaaccggatcaccatgtgcagcattcattggagatgacaatatcgtgaaaggagtcaaatcggacaaattaatggcagacaggtgcgccacctggttgaatatggaagtcaagattatagatgctgtggtgggcgagaaagcgccttatttctgtggagggtttattttgtgtgactccgtgaccggcacagcgtgccgtgtggcagaccccctaaaaaggctgtttaagctaggcaaacctctggcagcagacgatgaacatgatgatgacaggagaagggcattgcatgaggagtcaacacgctggaaccgagtgggtattctttcagagctgtgcaaggcagtagaatcaaggtatgaaaccgtaggaacttccatcatagttatggccatgactactctagctagcagtgttaaatcattcagctacctgagaggggcccctataactctctacggctaacctgaatggactacgacatagtctagtccgccaagactagtatgttcgtgttcctggtgctgctgcctctggtgtccagccagtgtgtgaacctgaccaccagaacacagctgcctccagcctacaccaacagctttaccagaggcgtgtactaccccgacaaggtgttcagatccagcgtgctgcactctacccaggacctgttcctgcctttcttcagcaacgtgacctggttccacgccatccacgtgtccggcaccaatggcaccaagagattcgacaaccccgtgctgcccttcaacgacggggtgtactttgccagcaccgagaagtccaacatcatcagaggctggatcttcggcaccacactggacagcaagacccagagcctgctgatcgtgaacaacgccaccaacgtggtcatcaaagtgtgcgagttccagttctgcaacgaccccttcctgggcgtctactaccacaagaacaacaagagctggatggaaagcgagttccgggtgtacagcagcgccaacaactgcaccttcgagtacgtgtcccagcctttcctgatggacctggaaggcaagcagggcaacttcaagaacctgcgcgagttcgtgtttaagaacatcgacggctacttcaagatctacagcaagcacacccctatcaacctcgtgcgggatctgcctcagggcttctctgctctggaacccctggtggatctgcccatcggcatcaacatcacccggtttcagacactgctggccctgcacagaagctacctgacacctggcgatagcagcagcggatggacagctggtgccgccgcttactatgtgggctacctgcagcctagaaccttcctgctgaagtacaacgagaacggcaccatcaccgacgccgtggattgtgctctggatcctctgagcgagacaaagtgcaccctgaagtccttcaccgtggaaaagggcatctaccagaccagcaacttccgggtgcagcccaccgaatccatcgtgcggttccccaatatcaccaatctgtgccccttcggcgaggtgttcaatgccaccagattcgcctctgtgtacgcctggaaccggaagcggatcagcaattgcgtggccgactactccgtgctgtacaactccgccagcttcagcaccttcaagtgctacggcgtgtcccctaccaagctgaacgacctgtgcttcacaaacgtgtacgccgacagcttcgtgatccggggagatgaagtgcggcagattgcccctggacagacaggcaagatcgccgactacaactacaagctgcccgacgacttcaccggctgtgtgattgcctggaacagcaacaacctggactccaaagtcggcggcaactacaattacctgtaccggctgttccggaagtccaatctgaagcccttcgagcgggacatctccaccgagatctatcaggccggcagcaccccttgtaacggcgtggaaggcttcaactgctacttcccactgcagtcctacggctttcagcccacaaatggcgtgggctatcagccctacagagtggtggtgctgagcttcgaactgctgcatgcccctgccacagtgtgcggccctaagaaaagcaccaatctcgtgaagaacaaatgcgtgaacttcaacttcaacggcctgaccggcaccggcgtgctgacagagagcaacaagaagttcctgccattccagcagtttggccgggatatcgccgataccacagacgccgttagagatccccagacactggaaatcctggacatcaccccttgcagcttcggcggagtgtctgtgatcacccctggcaccaacaccagcaatcaggtggcagtgctgtaccaggacgtgaactgtaccgaagtgcccgtggccattcacgccgatcagctgacacctacatggcgggtgtactccaccggcagcaatgtgtttcagaccagagccggctgtctgatcggagccgagcacgtgaacaatagctacgagtgcgacatccccatcggcgctggaatctgcgccagctaccagacacagacaaacagccctcggagagccagaagcgtggccagccagagcatcattgcctacacaatgtctctgggcgccgagaacagcgtggcctactccaacaactctatcgctatccccaccaacttcaccatcagcgtgaccacagagatcctgcctgtgtccatgaccaagaccagcgtggactgcaccatgtacatctgcggcgattccaccgagtgctccaacctgctgctgcagtacggcagcttctgcacccagctgaatagagccctgacagggatcgccgtggaacaggacaagaacacccaagaggtgttcgcccaagtgaagcagatctacaagacccctcctatcaaggacttcggcggcttcaatttcagccagattctgcccgatcctagcaagcccagcaagcggagcttcatcgaggacctgctgttcaacaaagtgacactggccgacgccggcttcatcaagcagtatggcgattgtctgggcgacattgccgccagggatctgatttgcgcccagaagtttaacggactgacagtgctgcctcctctgctgaccgatgagatgatcgcccagtacacatctgccctgctggccggcacaatcacaagcggctggacatttggagcaggcgccgctctgcagatcccctttgctatgcagatggcctaccggttcaacggcatcggagtgacccagaatgtgctgtacgagaaccagaagctgatcgccaaccagttcaacagcgccatcggcaagatccaggacagcctgagcagcacagcaagcgccctgggaaagctgcaggacgtggtcaaccagaatgcccaggcactgaacaccctggtcaagcagctgtcctccaacttcggcgccatcagctctgtgctgaacgatatcctgagcagactggaccctcctgaggccgaggtgcagatcgacagactgatcacaggcagactgcagagcctccagacatacgtgacccagcagctgatcagagccgccgagattagagcctctgccaatctggccgccaccaagatgtctgagtgtgtgctgggccagagcaagagagtggacttttgcggcaagggctaccacctgatgagcttccctcagtctgcccctcacggcgtggtgtttctgcacgtgacatatgtgcccgctcaagagaagaatttcaccaccgctccagccatctgccacgacggcaaagcccactttcctagagaaggcgtgttcgtgtccaacggcacccattggttcgtgacacagcggaacttctacgagccccagatcatcaccaccgacaacaccttcgtgtctggcaactgcgacgtcgtgatcggcattgtgaacaataccgtgtacgaccctctgcagcccgagctggacagcttcaaagaggaactggacaagtactttaagaaccacacaagccccgacgtggacctgggcgatatcagcggaatcaatgccagcgtcgtgaacatccagaaagagatcgaccggctgaacgaggtggccaagaatctgaacgagagcctgatcgacctgcaagaactggggaagtacgagcagtacatcaagtggccctggtacatctggctgggctttatcgccggactgattgccatcgtgatggtcacaatcatgctgtgttgcatgaccagctgctgtagctgcctgaagggctgttgtagctgtggcagctgctgcaagttcgacgaggacgattctgagcccgtgctgaagggcgtgaaactgcactacacatgatgactcgagctggtactgcatgcacgcaatgctagctgcccctttcccgtcctgggtaccccgagtctcccccgacctcgggtcccaggtatgctcccacctccacctgccccactcaccacctctgctagttccagacacctcccaagcacgcagcaatgcagctcaaaacgcttagcctagccacacccccacgggaaacagcagtgattaacctttagcaataaacgaaagtttaactaagctatactaaccccagggttggtcaatttcgtgccagccacaccgcggccgcatgaatacagcagcaattggcaagctgcttacatagaactcgcggcgattggcatgccgccttaaaatttttattttattttttcttttcttttccgaatcggattttgtttttaatatttcaaaaaaaaaaaaaaaaaaaaaaaaaaaaaagcatatgactaaaaaaaaaaaaaaaaaaaaaaaaaaaaaaaaaaaaaaaaaaaaaaaaaaaaaaaaaaaaaaaaaaaaaa

SEQ ID NO: 35 - RNA, 8896 nt, synthetic construct
  misc_feature 1..8896: note = Description of Artificial Sequence: Synthetic polynucleotide
  source 1..8896: mol_type = other RNA
gatgggcggcgcatgagagaagcccagaccaattacctacccaaaatggagaaagttcacgttgacatcgaggaagacagcccattcctcagagctttgcagcggagcttcccgcagtttgaggtagaagccaagcaggtcactgataatgaccatgctaatgccagagcgttttcgcatctggcttcaaaactgatcgaaacggaggtggacccatccgacacgatccttgacattggaagtgcgcccgcccgcagaatgtattctaagcacaagtatcattgtatctgtccgatgagatgtgcggaagatccggacagattgtataagtatgcaactaagctgaagaaaaactgtaaggaaataactgataaggaattggacaagaaaatgaaggagctcgccgccgtcatgagcgaccctgacctggaaactgagactatgtgcctccacgacgacgagtcgtgtcgctacgaagggcaagtcgctgtttaccaggatgtatacgcggttgacggaccgacaagtctctatcaccaagccaataagggagttagagtcgcctactggataggctttgacaccaccccttttatgtttaagaacttggctggagcatatccatcatactctaccaactgggccgacgaaaccgtgttaacggctcgtaacataggcctatgcagctctgacgttatggagcggtcacgtagagggatgtccattcttagaaagaagtatttgaaaccatccaacaatgttctattctctgttggctcgaccatctaccacgaaaagagggacttactgaggagctggcacctgccgtctgtatttcacttacgtggcaagcaaaattacacatgtcggtgtgagactatagttagttgcgacgggtacgtcgttaaaagaatagctatcagtccaggcctgtatgggaagccttcaggctatgctgctacgatgcaccgcgagggattcttgtgctgcaaagtgacagacacattgaacggggagagggtctcttttcccgtgtgcacgtatgtgccagctacattgtgtgaccaaatgactggcatactggcaacagatgtcagtgcggacgacgcgcaaaaactgctggttgggctcaaccagcgtatagtcgtcaacggtcgcacccagagaaacaccaataccatgaaaaattaccttttgcccgtagtggcccaggcatttgctaggtgggcaaaggaatataaggaagatcaagaagatgaaaggccactaggactacgagatagacagttagtcatggggtgttgttgggcttttagaaggcacaagataacatctatttataagcgcccggatacccaaaccatcatcaaagtgaacagcgatttccactcattcgtgctgcccaggataggcagtaacacattggagatcgggctgagaacaagaatcaggaaaatgttagaggagcacaaggagccgtcacctctcattaccgccgaggacgtacaagaagctaagtgcgcagccgatgaggctaaggaggtgcgtgaagccgaggagttgcgcgcagctctaccacctttggcagctgatgttgaggagcccactctggaagccgatgtcgacttgatgttacaagaggctggggccggctcagtggagacacctcgtggcttgataaaggttaccagctacgctggcgaggacaagatcggctcttacgctgtgctttctccgcaggctgtactcaagagtgaaaaattatcttgcatccaccctctcgctgaacaagtcatagtgataacacactctggccgaaaagggcgttatgccgtggaaccataccatggtaaagtagtggtgccagagggacatgcaatacccgtccaggactttcaagctctgagtgaaagtgccaccattgtgtacaacgaacgtgagttcgtaaacaggtacctgcaccatattgccacacatggaggagcgctgaacactgatgaagaatattacaaaactgtcaagcccagcgagcacgacggcgaatacctgtacgacatcgacaggaaacagtgcgtcaagaaagagctagtcactgggctagggctcacaggcgagctggtcgatcctcccttccatgaattcgcctacgagagtctgagaacacgaccagccgctccttaccaagtaccaaccataggggtgtatggcgtgccaggatcaggcaagtctggcatcattaaaagcgcagtcaccaaaaaagatctagtggtgagcgccaagaaagaaaactgtgcagaaattataagggacgtcaagaaaatgaaagggctggacgtcaatgccagaactgtggactcagtgctcttgaatggatgcaaacaccccgtagagaccctgtatattgacgaggcttttgcttgtcatgcaggtactctcagagcgctcatagccattataagacctaaaaaggcagtgctctgcggagatcccaaacagtgcggtttttttaacatgatgtgcctgaaagtgcattttaaccacgagatttgcacacaagtcttccacaaaagcatctctcgccgttgcactaaatctgtgacttcggtcgtctcaaccttgttttacgacaaaaaaatgagaacgacgaatccgaaagagactaagattgtgattgacactaccggcagtaccaaacctaagcaggacgatctcattctcacttgtttcagagggtgggtgaagcagttgcaaatagattacaaaggcaacgaaataatgacggcagctgcctctcaagggctgacccgtaaaggtgtgtatgccgttcggtacaaggtgaatgaaaatcctctgtacgcacccacctcagaacatgtgaacgtcctactgacccgcacggaggaccgcatcgtgtggaaaacactagccggcgacccatggataaaaacactgactgccaagtaccctgggaatttcactgccacgatagaggagtggcaagcagagcatgatgccatcatgaggcacatcttggagagaccggaccctaccgacgtcttccagaataaggcaaacgtgtgttgggccaaggctttagtgccggtgctgaagaccgctggcatagacatgaccactgaacaatggaacactgtggattattttgaaacggacaaagctcactcagcagagatagtattgaaccaactatgcgtgaggttctttggactcgatctggactccggtctattttctgcacccactgttccgttatccattaggaataatcactgggataactccccgtcgcctaacatgtacgggctgaataaagaagtggtccgtcagctctctcgcaggtacccacaactgcctcgggcagttgccactggtagagtctatgacatgaacactggtacactgcgcaattatgatccgcgcataaacctagtacctgtaaacagaagactgcctcatgctttagtcctccaccataatgaacacccacagagtgacttttcttcattcgtcagcaaattgaagggcagaactgtcctggtggtcggggaaaagttgtccgtcccaggcaaaatggttgactggttgtcagaccggcctgaggctaccttcagagctcggctggatttaggcatcccaggtgatgtgcccaaatatgacataatatttgttaatgtgaggaccccatataaataccatcactatcagcagtgtgaagaccatgccattaagctaagcatgttgaccaagaaagcatgtctgcatctgaatcccggcggaacctgtgtcagcataggttatggttacgctgacagggccagcgaaagcatcattggtgctatagcgcggcagttcaagttttcccgagtatgcaaaccgaaatcctcacttgaggagacggaagttctgtttgtattcattgggtacgatcgcaaggcccgtacgcacaatccttacaagctatcatcaaccttgaccaacatttatacaggttccagactccacgaagccggatgtgcaccctcatatcatgtggtgcgaggggatattgccacggccaccgaaggagtgattataaatgctgctaacagcaaaggacaacctggcggaggggtgtgcggagcgctgtataagaaattcccggaaagtttcgatttacagccgatcgaagtaggaaaagcgcgactggtcaaaggtgcagctaaacatatcattcatgccgtaggaccaaacttcaacaaagtttcggaggttgaaggtgacaaacagttggcagaggcttatgagtccatcgctaagattgtcaacgataacaattacaagtcagtagcgattccactgttgtccaccggcatcttttccgggaacaaagatcgactaacccaatcattgaaccatttgctgacagctttagacaccactgatgcagatgtagccatatactgcagggacaagaaatgggaaatgactctcaaggaagcagtggctaggagagaagcagtggaggagatatgcatatccgacgattcttcagtgacagaacctgatgcagagctggtgagggtgcatcccaagagttctttggctggaaggaagggctacagcacaagcgatggcaaaactttctcatatttggaagggaccaagtttcaccaggcggccaaggatatagcagaaattaatgccatgtggcccgttgcaacggaggccaatgagcaggtatgcatgtatatcctcggagaaagcatgagcagtattaggtcgaaatgccccgtcgaggagtcggaagcctccacaccacctagcacgctgccttgcttgtgcatccatgccatgactccagaaagagtacagcgcctaaaagcctcacgtccagaacaaattactgtgtgctcatcctttccattgccgaagtatagaatcactggtgtgcagaagatccaatgctcccagcctatattgttctcaccgaaagtgcctgcgtatattcatccaaggaagtatctcgtggaaacaccaccggtagacgagactccggagccatcggcagagaaccaatccacagaggggacacctgaacaaccaccacttataaccgaggatgagaccaggactagaacgcctgagccgatcatcatcgaagaagaagaagaagatagcataagtttgctgtcagatggcccgacccaccaggtgctgcaagtcgaggcagacattcacgggccgccctctgtatctagctcatcctggtccattcctcatgcatccgactttgatgtggacagtttatccatacttgacaccctggagggagctagcgtgaccagcggggcaacgtcagccgagactaactcttacttcgcaaagagtatggagtttctggcgcgaccggtgcctgcgcctcgaacagtattcaggaaccctccacatcccgctccgcgcacaagaacaccgtcacttgcacccagcagggcctgctccagaaccagcctagtttccaccccgccaggcgtgaatagggtgatcactagagaggagctcgaagcgcttaccccgtcacgcactcctagcaggtcggtctccagaaccagcctggtctccaacccgccaggcgtaaatagggtgattacaagagaggagtttgaggcgttcgtagcacaacaacaatgacggtttgatgcgggtgcatacatcttttcctccgacaccggtcaagggcatttacaacaaaaatcagtaaggcaaacggtgctatccgaagtggtgttggagaggaccgaattggagatttcgtatgccccgcgcctcgaccaagaaaaagaagaattactacgcaagaaattacagttaaatcccacacctgctaacagaagcagataccagtccaggaaggtggagaacatgaaagccataacagctagacgtattctgcaaggcctagggcattatttgaaggcagaaggaaaagtggagtgctaccgaaccctgcatcctgttcctttgtattcatctagtgtgaaccgtgccttttcaagccccaaggtcgcagtggaagcctgtaacgccatgttgaaagagaactttccgactgtggcttcttactgtattattccagagtacgatgcctatttggacatggttgacggagcttcatgctgcttagacactgccagtttttgccctgcaaagctgcgcagctttccaaagaaacactcctatttggaacccacaatacgatcggcagtgccttcagcgatccagaacacgctccagaacgtcctggcagctgccacaaaaagaaattgcaatgtcacgcaaatgagagaattgcccgtattggattcggcggcctttaatgtggaatgcttcaagaaatatgcgtgtaataatgaatattgggaaacgtttaaagaaaaccccatcaggcttactgaagaaaacgtggtaaattacattaccaaattaaaaggaccaaaagctgctgctctttttgcgaagacacataatttgaatatgttgcaggacataccaatggacaggtttgtaatggacttaaagagagacgtgaaagtgactccaggaacaaaacatactgaagaacggcccaaggtacaggtgatccaggctgccgatccgctagcaacagcgtatctgtgcggaatccaccgagagctggttaggagattaaatgcggtcctgcttccgaacattcatacactgtttgatatgtcggctgaagactttgacgctattatagccgagcacttccagcctggggattgtgttctggaaactgacatcgcgtcgtttgataaaagtgaggacgacgccatggctctgaccgcgttaatgattctggaagacttaggtgtggacgcagagctgttgacgctgattgaggcggctttcggcgaaatttcatcaatacatttgcccactaaaactaaatttaaattcggagccatgatgaaatctggaatgttcctcacactgtttgtgaacacagtcattaacattgtaatcgcaagcagagtgttgagagaacggctaaccggatcaccatgtgcagcattcattggagatgacaatatcgtgaaaggagtcaaatcggacaaattaatggcagacaggtgcgccacctggttgaatatggaagtcaagattatagatgctgtggtgggcgagaaagcgccttatttctgtggagggtttattttgtgtgactccgtgaccggcacagcgtgccgtgtggcagaccccctaaaaaggctgtttaagctaggcaaacctctggcagcagacgatgaacatgatgatgacaggagaagggcattgcatgaggagtcaacacgctggaaccgagtgggtattctttcagagctgtgcaaggcagtagaatcaaggtatgaaaccgtaggaacttccatcatagttatggccatgactactctagctagcagtgttaaatcattcagctacctgagaggggcccctataactctctacggctaacctgaatggactacgacatagtctagtccgccaagactagtatgtttgtgtttcttgtgctgctgcctcttgtgtcttctcagtgtgtggtgagatttccaaatattacaaatctgtgtccatttggagaagtgtttaatgcaacaagatttgcatctgtgtatgcatggaatagaaaaagaatttctaattgtgtggctgattattctgtgctgtataatagtgcttctttttccacatttaaatgttatggagtgtctccaacaaaattaaatgatttatgttttacaaatgtgtatgctgattcttttgtgatcagaggtgatgaagtgagacagattgcccccggacagacaggaaaaattgctgattacaattacaaactgcctgatgattttacaggatgtgtgattgcttggaattctaataatttagattctaaagtgggaggaaattacaattatctgtacagactgtttagaaaatcaaatctgaaaccttttgaaagagatatttcaacagaaatttatcaggctggatcaacaccttgtaatggagtggaaggatttaattgttattttccattacagagctatggatttcagccaaccaatggtgtgggatatcagccatatagagtggtggtgctgtcttttgaactgctgcatgcacctgcaacagtgtgtggacctaaaggctcccccggctccggctccggatctggttatattcctgaagctccaagagatgggcaagcttacgttcgtaaagatggcgaatgggtattactttctacctttttaggccggtccctggaggtgctgttccagggccccggctgatgactcgagctggtactgcatgcacgcaatgctagctgcccctttcccgtcctgggtaccccgagtctcccccgacctcgggtcccaggtatgctcccacctccacctgccccactcaccacctctgctagttccagacacctcccaagcacgcagcaatgcagctcaaaacgcttagcctagccacacccccacgggaaacagcagtgattaacctttagcaataaacgaaagtttaactaagctatactaaccccagggttggtcaatttcgtgccagccacaccgcggccgcatgaatacagcagcaattggcaagctgcttacatagaactcgcggcgattggcatgccgccttaaaatttttattttattttttcttttcttttccgaatcggattttgtttttaatatttcaaaaaaaaaaaaaaaaaaaaaaaaaaaaaagcatatgactaaaaaaaaaaaaaaaaaaaaaaaaaaaaaaaaaaaaaaaaaaaaaaaaaaaaaaaaaaaaaaaaaaaaaa

SEQ ID NO: 36 - RNA, 9079 nt, synthetic construct
  misc_feature 1..9079: note = Description of Artificial Sequence: Synthetic polynucleotide
  source 1..9079: mol_type = other RNA
gatgggcggcgcatgagagaagcccagaccaattacctacccaaaatggagaaagttcacgttgacatcgaggaagacagcccattcctcagagctttgcagcggagcttcccgcagtttgaggtagaagccaagcaggtcactgataatgaccatgctaatgccagagcgttttcgcatctggcttcaaaactgatcgaaacggaggtggacccatccgacacgatccttgacattggaagtgcgcccgcccgcagaatgtattctaagcacaagtatcattgtatctgtccgatgagatgtgcggaagatccggacagattgtataagtatgcaactaagctgaagaaaaactgtaaggaaataactgataaggaattggacaagaaaatgaaggagctcgccgccgtcatgagcgaccctgacctggaaactgagactatgtgcctccacgacgacgagtcgtgtcgctacgaagggcaagtcgctgtttaccaggatgtatacgcggttgacggaccgacaagtctctatcaccaagccaataagggagttagagtcgcctactggataggctttgacaccaccccttttatgtttaagaacttggctggagcatatccatcatactctaccaactgggccgacgaaaccgtgttaacggctcgtaacataggcctatgcagctctgacgttatggagcggtcacgtagagggatgtccattcttagaaagaagtatttgaaaccatccaacaatgttctattctctgttggctcgaccatctaccacgaaaagagggacttactgaggagctggcacctgccgtctgtatttcacttacgtggcaagcaaaattacacatgtcggtgtgagactatagttagttgcgacgggtacgtcgttaaaagaatagctatcagtccaggcctgtatgggaagccttcaggctatgctgctacgatgcaccgcgagggattcttgtgctgcaaagtgacagacacattgaacggggagagggtctcttttcccgtgtgcacgtatgtgccagctacattgtgtgaccaaatgactggcatactggcaacagatgtcagtgcggacgacgcgcaaaaactgctggttgggctcaaccagcgtatagtcgtcaacggtcgcacccagagaaacaccaataccatgaaaaattaccttttgcccgtagtggcccaggcatttgctaggtgggcaaaggaatataaggaagatcaagaagatgaaaggccactaggactacgagatagacagttagtcatggggtgttgttgggcttttagaaggcacaagataacatctatttataagcgcccggatacccaaaccatcatcaaagtgaacagcgatttccactcattcgtgctgcccaggataggcagtaacacattggagatcgggctgagaacaagaatcaggaaaatgttagaggagcacaaggagccgtcacctctcattaccgccgaggacgtacaagaagctaagtgcgcagccgatgaggctaaggaggtgcgtgaagccgaggagttgcgcgcagctctaccacctttggcagctgatgttgaggagcccactctggaagccgatgtcgacttgatgttacaagaggctggggccggctcagtggagacacctcgtggcttgataaaggttaccagctacgctggcgaggacaagatcggctcttacgctgtgctttctccgcaggctgtactcaagagtgaaaaattatcttgcatccaccctctcgctgaacaagtcatagtgataacacactctggccgaaaagggcgttatgccgtggaaccataccatggtaaagtagtggtgccagagggacatgcaatacccgtccaggactttcaagctctgagtgaaagtgccaccattgtgtacaacgaacgtgagttcgtaaacaggtacctgcaccatattgccacacatggaggagcgctgaacactgatgaagaatattacaaaactgtcaagcccagcgagcacgacggcgaatacctgtacgacatcgacaggaaacagtgcgtcaagaaagagctagtcactgggctagggctcacaggcgagctggtcgatcctcccttccatgaattcgcctacgagagtctgagaacacgaccagccgctccttaccaagtaccaaccataggggtgtatggcgtgccaggatcaggcaagtctggcatcattaaaagcgcagtcaccaaaaaagatctagtggtgagcgccaagaaagaaaactgtgcagaaattataagggacgtcaagaaaatgaaagggctggacgtcaatgccagaactgtggactcagtgctcttgaatggatgcaaacaccccgtagagaccctgtatattgacgaggcttttgcttgtcatgcaggtactctcagagcgctcatagccattataagacctaaaaaggcagtgctctgcggagatcccaaacagtgcggtttttttaacatgatgtgcctgaaagtgcattttaaccacgagatttgcacacaagtcttccacaaaagcatctctcgccgttgcactaaatctgtgacttcggtcgtctcaaccttgttttacgacaaaaaaatgagaacgacgaatccgaaagagactaagattgtgattgacactaccggcagtaccaaacctaagcaggacgatctcattctcacttgtttcagagggtgggtgaagcagttgcaaatagattacaaaggcaacgaaataatgacggcagctgcctctcaagggctgacccgtaaaggtgtgtatgccgttcggtacaaggtgaatgaaaatcctctgtacgcacccacctcagaacatgtgaacgtcctactgacccgcacggaggaccgcatcgtgtggaaaacactagccggcgacccatggataaaaacactgactgccaagtaccctgggaatttcactgccacgatagaggagtggcaagcagagcatgatgccatcatgaggcacatcttggagagaccggaccctaccgacgtcttccagaataaggcaaacgtgtgttgggccaaggctttagtgccggtgctgaagaccgctggcatagacatgaccactgaacaatggaacactgtggattattttgaaacggacaaagctcactcagcagagatagtattgaaccaactatgcgtgaggttctttggactcgatctggactccggtctattttctgcacccactgttccgttatccattaggaataatcactgggataactccccgtcgcctaacatgtacgggctgaataaagaagtggtccgtcagctctctcgcaggtacccacaactgcctcgggcagttgccactggtagagtctatgacatgaacactggtacactgcgcaattatgatccgcgcataaacctagtacctgtaaacagaagactgcctcatgctttagtcctccaccataatgaacacccacagagtgacttttcttcattcgtcagcaaattgaagggcagaactgtcctggtggtcggggaaaagttgtccgtcccaggcaaaatggttgactggttgtcagaccggcctgaggctaccttcagagctcggctggatttaggcatcccaggtgatgtgcccaaatatgacataatatttgttaatgtgaggaccccatataaataccatcactatcagcagtgtgaagaccatgccattaagctaagcatgttgaccaagaaagcatgtctgcatctgaatcccggcggaacctgtgtcagcataggttatggttacgctgacagggccagcgaaagcatcattggtgctatagcgcggcagttcaagttttcccgagtatgcaaaccgaaatcctcacttgaggagacggaagttctgtttgtattcattgggtacgatcgcaaggcccgtacgcacaatccttacaagctatcatcaaccttgaccaacatttatacaggttccagactccacgaagccggatgtgcaccctcatatcatgtggtgcgaggggatattgccacggccaccgaaggagtgattataaatgctgctaacagcaaaggacaacctggcggaggggtgtgcggagcgctgtataagaaattcccggaaagtttcgatttacagccgatcgaagtaggaaaagcgcgactggtcaaaggtgcagctaaacatatcattcatgccgtaggaccaaacttcaacaaagtttcggaggttgaaggtgacaaacagttggcagaggcttatgagtccatcgctaagattgtcaacgataacaattacaagtcagtagcgattccactgttgtccaccggcatcttttccgggaacaaagatcgactaacccaatcattgaaccatttgctgacagctttagacaccactgatgcagatgtagccatatactgcagggacaagaaatgggaaatgactctcaaggaagcagtggctaggagagaagcagtggaggagatatgcatatccgacgattcttcagtgacagaacctgatgcagagctggtgagggtgcatcccaagagttctttggctggaaggaagggctacagcacaagcgatggcaaaactttctcatatttggaagggaccaagtttcaccaggcggccaaggatatagcagaaattaatgccatgtggcccgttgcaacggaggccaatgagcaggtatgcatgtatatcctcggagaaagcatgagcagtattaggtcgaaatgccccgtcgaggagtcggaagcctccacaccacctagcacgctgccttgcttgtgcatccatgccatgactccagaaagagtacagcgcctaaaagcctcacgtccagaacaaattactgtgtgctcatcctttccattgccgaagtatagaatcactggtgtgcagaagatccaatgctcccagcctatattgttctcaccgaaagtgcctgcgtatattcatccaaggaagtatctcgtggaaacaccaccggtagacgagactccggagccatcggcagagaaccaatccacagaggggacacctgaacaaccaccacttataaccgaggatgagaccaggactagaacgcctgagccgatcatcatcgaagaagaagaagaagatagcataagtttgctgtcagatggcccgacccaccaggtgctgcaagtcgaggcagacattcacgggccgccctctgtatctagctcatcctggtccattcctcatgcatccgactttgatgtggacagtttatccatacttgacaccctggagggagctagcgtgaccagcggggcaacgtcagccgagactaactcttacttcgcaaagagtatggagtttctggcgcgaccggtgcctgcgcctcgaacagtattcaggaaccctccacatcccgctccgcgcacaagaacaccgtcacttgcacccagcagggcctgctccagaaccagcctagtttccaccccgccaggcgtgaatagggtgatcactagagaggagctcgaagcgcttaccccgtcacgcactcctagcaggtcggtctccagaaccagcctggtctccaacccgccaggcgtaaatagggtgattacaagagaggagtttgaggcgttcgtagcacaacaacaatgacggtttgatgcgggtgcatacatcttttcctccgacaccggtcaagggcatttacaacaaaaatcagtaaggcaaacggtgctatccgaagtggtgttggagaggaccgaattggagatttcgtatgccccgcgcctcgaccaagaaaaagaagaattactacgcaagaaattacagttaaatcccacacctgctaacagaagcagataccagtccaggaaggtggagaacatgaaagccataacagctagacgtattctgcaaggcctagggcattatttgaaggcagaaggaaaagtggagtgctaccgaaccctgcatcctgttcctttgtattcatctagtgtgaaccgtgccttttcaagccccaaggtcgcagtggaagcctgtaacgccatgttgaaagagaactttccgactgtggcttcttactgtattattccagagtacgatgcctatttggacatggttgacggagcttcatgctgcttagacactgccagtttttgccctgcaaagctgcgcagctttccaaagaaacactcctatttggaacccacaatacgatcggcagtgccttcagcgatccagaacacgctccagaacgtcctggcagctgccacaaaaagaaattgcaatgtcacgcaaatgagagaattgcccgtattggattcggcggcctttaatgtggaatgcttcaagaaatatgcgtgtaataatgaatattgggaaacgtttaaagaaaaccccatcaggcttactgaagaaaacgtggtaaattacattaccaaattaaaaggaccaaaagctgctgctctttttgcgaagacacataatttgaatatgttgcaggacataccaatggacaggtttgtaatggacttaaagagagacgtgaaagtgactccaggaacaaaacatactgaagaacggcccaaggtacaggtgatccaggctgccgatccgctagcaacagcgtatctgtgcggaatccaccgagagctggttaggagattaaatgcggtcctgcttccgaacattcatacactgtttgatatgtcggctgaagactttgacgctattatagccgagcacttccagcctggggattgtgttctggaaactgacatcgcgtcgtttgataaaagtgaggacgacgccatggctctgaccgcgttaatgattctggaagacttaggtgtggacgcagagctgttgacgctgattgaggcggctttcggcgaaatttcatcaatacatttgcccactaaaactaaatttaaattcggagccatgatgaaatctggaatgttcctcacactgtttgtgaacacagtcattaacattgtaatcgcaagcagagtgttgagagaacggctaaccggatcaccatgtgcagcattcattggagatgacaatatcgtgaaaggagtcaaatcggacaaattaatggcagacaggtgcgccacctggttgaatatggaagtcaagattatagatgctgtggtgggcgagaaagcgccttatttctgtggagggtttattttgtgtgactccgtgaccggcacagcgtgccgtgtggcagaccccctaaaaaggctgtttaagctaggcaaacctctggcagcagacgatgaacatgatgatgacaggagaagggcattgcatgaggagtcaacacgctggaaccgagtgggtattctttcagagctgtgcaaggcagtagaatcaaggtatgaaaccgtaggaacttccatcatagttatggccatgactactctagctagcagtgttaaatcattcagctacctgagaggggcccctataactctctacggctaacctgaatggactacgacatagtctagtccgccaagactagtatgtttgtgtttcttgtgctgctgcctcttgtgtcttctcagtgtgtggtgagatttccaaatattacaaatctgtgtccatttggagaagtgtttaatgcaacaagatttgcatctgtgtatgcatggaatagaaaaagaatttctaattgtgtggctgattattctgtgctgtataatagtgcttctttttccacatttaaatgttatggagtgtctccaacaaaattaaatgatttatgttttacaaatgtgtatgctgattcttttgtgatcagaggtgatgaagtgagacagattgcccccggacagacaggaaaaattgctgattacaattacaaactgcctgatgattttacaggatgtgtgattgcttggaattctaataatttagattctaaagtgggaggaaattacaattatctgtacagactgtttagaaaatcaaatctgaaaccttttgaaagagatatttcaacagaaatttatcaggctggatcaacaccttgtaatggagtggaaggatttaattgttattttccattacagagctatggatttcagccaaccaatggtgtgggatatcagccatatagagtggtggtgctgtcttttgaactgctgcatgcacctgcaacagtgtgtggacctaaaggctcccccggctccggctccggatctggttatattcctgaagctccaagagatgggcaagcttacgttcgtaaagatggcgaatgggtattactttctacctttttaggaagcggcagcggatctgaacagtacattaaatggccttggtacatttggcttggatttattgcaggattaattgcaattgtgatggtgacaattatgttatgttgtatgacatcatgttgttcttgtttaaaaggatgttgttcttgtggaagctgttgtaaatttgatgaagatgattctgaacctgtgttaaaaggagtgaaattgcattacacatgatgactcgagctggtactgcatgcacgcaatgctagctgcccctttcccgtcctgggtaccccgagtctcccccgacctcgggtcccaggtatgctcccacctccacctgccccactcaccacctctgctagttccagacacctcccaagcacgcagcaatgcagctcaaaacgcttagcctagccacacccccacgggaaacagcagtgattaacctttagcaataaacgaaagtttaactaagctatactaaccccagggttggtcaatttcgtgccagccacaccgcggccgcatgaatacagcagcaattggcaagctgcttacatagaactcgcggcgattggcatgccgccttaaaatttttattttattttttcttttcttttccgaatcggattttgtttttaatatttcaaaaaaaaaaaaaaaaaaaaaaaaaaaaaagcatatgactaaaaaaaaaaaaaaaaaaaaaaaaaaaaaaaaaaaaaaaaaaaaaaaaaaaaaaaaaaaaaaaaaaaaaa

SEQ ID NO: 37 - protein, 327 aa, synthetic construct
  REGION 1..327: note = Description of Artificial Sequence: Synthetic polypeptide
MFVFLVLLPLVSSQCVVRFPNITNLCPFGEVFNATRFASVYAWNRKRISNCVADYSVLYNSASFSTFKCYGVSPTKLNDLCFTNVYADSFVIRGDEVRQIAPGQTGKIADYNYKLPDDFTGCVIAWNSNNLDSKVGGNYNYLYRLFRKSNLKPFERDISTEIYQAGSTPCNGVEGFNCYFPLQSYGFQPTNGVGYQPYRVVVLSFELLHAPATVCGPKGSPGSGSGSGYIPEAPRDGQAYVRKDGEWVLLSTFLGSGSGSEQYIKWPWYIWLGFIAGLIAIVMVTIMLCCMTSCCSCLKGCCSCGSCCKFDEDDSEPVLKGVKLHYT

SEQ ID NO: 38 - protein, 311 aa, synthetic construct
  REGION 1..311: note = Description of Artificial Sequence: Synthetic polypeptide
MFVFLVLLPLVSSQCVNLTVRFPNITNLCPFGEVFNATRFASVYAWNRKRISNCVADYSVLYNSASFSTFKCYGVSPTKLNDLCFTNVYADSFVIRGDEVRQIAPGQTGKIADYNYKLPDDFTGCVIAWNSNNLDSKVGGNYNYLYRLFRKSNLKPFERDISTEIYQAGSTPCNGVEGFNCYFPLQSYGFQPTNGVGYQPYRVVVLSFELLHAPATVCGPKGSPGSGSGSGYIPEAPRDGQAYVRKDGEWVLLSTFLGSGSGSEQYIKWPWYIWLGFIAGLIAIVMVTIMLCCMTSCCSCLKGCCSCGSCC

SEQ ID NO: 39 - RNA, 1397 nt, synthetic construct
  misc_feature 1..1397: note = Description of Artificial Sequence: Synthetic polynucleotide
  source 1..1397: mol_type = other RNA
agaataaactagtattcttctggtccccacagactcagagagaacccgccaccatgtttgtgtttcttgtgctgctgcctcttgtgtcttctcagtgtgtgaatttgacagtgagatttccaaatattacaaatctgtgtccatttggagaagtgtttaatgcaacaagatttgcatctgtgtatgcatggaatagaaaaagaatttctaattgtgtggctgattattctgtgctgtataatagtgcttctttttccacatttaaatgttatggagtgtctccaacaaaattaaatgatttatgttttacaaatgtgtatgctgattcttttgtgatcagaggtgatgaagtgagacagattgcccccggacagacaggaaaaattgctgattacaattacaaactgcctgatgattttacaggatgtgtgattgcttggaattctaataatttagattctaaagtgggaggaaattacaattatctgtacagactgtttagaaaatcaaatctgaaaccttttgaaagagatatttcaacagaaatttatcaggctggatcaacaccttgtaatggagtggaaggatttaattgttattttccattacagagctatggatttcagccaaccaatggtgtgggatatcagccatatagagtggtggtgctgtcttttgaactgctgcatgcacctgcaacagtgtgtggacctaaaggctcccccggctccggctccggatctggttatattcctgaagctccaagagatgggcaagcttacgttcgtaaagatggcgaatgggtattactttctacctttttaggaagcggcagcggatctgaacagtacattaaatggccttggtacatttggcttggatttattgcaggattaattgcaattgtgatggtgacaattatgttatgttgtatgacatcatgttgttcttgtttaaaaggatgttgttcttgtggaagctgttgttgatgactcgagctggtactgcatgcacgcaatgctagctgcccctttcccgtcctgggtaccccgagtctcccccgacctcgggtcccaggtatgctcccacctccacctgccccactcaccacctctgctagttccagacacctcccaagcacgcagcaatgcagctcaaaacgcttagcctagccacacccccacgggaaacagcagtgattaacctttagcaataaacgaaagtttaactaagctatactaaccccagggttggtcaatttcgtgccagccacaccctggagctagcaaaaaaaaaaaaaaaaaaaaaaaaaaaaaagcatatgactaaaaaaaaaaaaaaaaaaaaaaaaaaaaaaaaaaaaaaaaaaaaaaaaaaaaaaaaaaaaaaaaaaaaaa

SEQ ID NO: 40 - protein, 314 aa, synthetic construct
  REGION 1..314: note = Description of Artificial Sequence: Synthetic polypeptide
MDWIWRILFLVGAATGAHSQMQVRFPNITNLCPFGEVFNATRFASVYAWNRKRISNCVADYSVLYNSASFSTFKCYGVSPTKLNDLCFTNVYADSFVIRGDEVRQIAPGQTGKIADYNYKLPDDFTGCVIAWNSNNLDSKVGGNYNYLYRLFRKSNLKPFERDISTEIYQAGSTPCNGVEGFNCYFPLQSYGFQPTNGVGYQPYRVVVLSFELLHAPATVCGPKGSPGSGSGSGYIPEAPRDGQAYVRKDGEWVLLSTFLGSGSGSEQYIKWPWYIWLGFIAGLIAIVMVTIMLCCMTSCCSCLKGCCSCGSCC

SEQ ID NO: 41 - RNA, 1406 nt, synthetic construct
  misc_feature 1..1406: note = Description of Artificial Sequence: Synthetic polynucleotide
  source 1..1406: mol_type = other RNA
agaataaactagtattcttctggtccccacagactcagagagaacccgccaccatggattggatttggagaatcctgttcctcgtgggagccgctacaggagcccactcccagatgcaggtgagatttccaaatattacaaatctgtgtccatttggagaagtgtttaatgcaacaagatttgcatctgtgtatgcatggaatagaaaaagaatttctaattgtgtggctgattattctgtgctgtataatagtgcttctttttccacatttaaatgttatggagtgtctccaacaaaattaaatgatttatgttttacaaatgtgtatgctgattcttttgtgatcagaggtgatgaagtgagacagattgcccccggacagacaggaaaaattgctgattacaattacaaactgcctgatgattttacaggatgtgtgattgcttggaattctaataatttagattctaaagtgggaggaaattacaattatctgtacagactgtttagaaaatcaaatctgaaaccttttgaaagagatatttcaacagaaatttatcaggctggatcaacaccttgtaatggagtggaaggatttaattgttattttccattacagagctatggatttcagccaaccaatggtgtgggatatcagccatatagagtggtggtgctgtcttttgaactgctgcatgcacctgcaacagtgtgtggacctaaaggctcccccggctccggctccggatctggttatattcctgaagctccaagagatgggcaagcttacgttcgtaaagatggcgaatgggtattactttctacctttttaggaagcggcagcggatctgaacagtacattaaatggccttggtacatttggcttggatttattgcaggattaattgcaattgtgatggtgacaattatgttatgttgtatgacatcatgttgttcttgtttaaaaggatgttgttcttgtggaagctgttgttgatgactcgagctggtactgcatgcacgcaatgctagctgcccctttcccgtcctgggtaccccgagtctcccccgacctcgggtcccaggtatgctcccacctccacctgccccactcaccacctctgctagttccagacacctcccaagcacgcagcaatgcagctcaaaacgcttagcctagccacacccccacgggaaacagcagtgattaacctttagcaataaacgaaagtttaactaagctatactaaccccagggttggtcaatttcgtgccagccacaccctggagctagcaaaaaaaaaaaaaaaaaaaaaaaaaaaaaagcatatgactaaaaaaaaaaaaaaaaaaaaaaaaaaaaaaaaaaaaaaaaaaaaaaaaaaaaaaaaaaaaaaaaaaaaaa

SEQ ID NO: 42 - DNA, 55 bp, synthetic construct
  misc_feature 1..55: note = Description of Artificial Sequence: Synthetic oligonucleotide
  misc_feature 1..55: note = Description of Combined DNA/RNA Molecule: Synthetic oligonucleotide
  source 1..55: mol_type = other DNA
  misc_feature 1..53: note = DNA
  misc_feature 54..55: note = RNA
agacgaactagtattcttctggtccccacagactcagagagaacccgccaccatg

SEQ ID NO: 43 - RNA, 15 nt, synthetic construct
  misc_feature 1..15: note = Description of Artificial Sequence: Synthetic oligonucleotide
  source 1..15: mol_type = other RNA
gctagccgcgtcgct

SEQ ID NO: 44 - RNA, 19 nt, synthetic construct
  misc_feature 1..19: note = Description of Artificial Sequence: Synthetic oligonucleotide
  source 1..19: mol_type = other RNA
atttacgaacgatagcatg

SEQ ID NO: 45 - DNA, 56 bp, synthetic construct
  misc_feature 1..56: note = Description of Artificial Sequence: Synthetic oligonucleotide
  misc_feature 1..56: note = Description of Combined DNA/RNA Molecule: Synthetic oligonucleotide
  source 1..56: mol_type = other DNA
  misc_feature 1..18: note = DNA
  misc_feature 19..56: note = RNA
agcacgcagcaatgcagctcaaaacgcttagcctagccacacccccacgggaaaca

SEQ ID NO: 46 - RNA, 20 nt, synthetic construct
  misc_feature 1..20: note = Description of Artificial Sequence: Synthetic oligonucleotide
  source 1..20: mol_type = other RNA
gagtcgctagccgcgtcgct